European Patent Application EP 4 311 862 A1, published January 31, 2024. Title: METHODS FOR DETECTION OF EMBRYO IMPLANTATION FAILURE OF ENDOMETRIAL ORIGEN. Applicant: IVI RMA GLOBAL, SL. Application EP, filed July 29, 2022. The sequence listing filed with the application follows.

SEQUENCE LISTING (760 sequences)

SEQ ID NO: 1 - DNA, 75 bp, Homo sapiens
  source 1..75: mol_type = genomic DNA
gggttttctgtgtgcacagacaggttggagtcccagaacttggagccgagctccccggaaccgcacagggcgtcc

SEQ ID NO: 2 - DNA, 65 bp, Homo sapiens
  source 1..65: mol_type = genomic DNA
aaaatcctgcccacgggttgacgaatcacccttccatattgagtcatgatcccaggagggaagta

SEQ ID NO: 3 - DNA, 75 bp, Homo sapiens
  source 1..75: mol_type = genomic DNA
tcctccatgttctccgtaaagtggtccaggtgctcaggaaagtgcgcattgttgaggaagtccgactcgttcaga

SEQ ID NO: 4 - DNA, 54 bp, Homo sapiens
  source 1..54: mol_type = genomic DNA
ggagttacaccatgccgtgaatgtctttctctgctgcttctcccaggccgggtc

SEQ ID NO: 5 - DNA, 72 bp, Homo sapiens
  source 1..72: mol_type = genomic DNA
ttttcccactcttggattcgtgccattcattgttgataaatatcttggtgaacttgacctccaggttgcgga

SEQ ID NO: 6 - DNA, 77 bp, Homo sapiens
  source 1..77: mol_type = genomic DNA
ttattagtagcttttctcttcatagttgctatattgccagctttttgtgtctgttgattcagtgaatccagaaactt

SEQ ID NO: 7 - DNA, 69 bp, Homo sapiens
  source 1..69: mol_type = genomic DNA
agagaatctgaatcaaattcccttgtgaatgttagatgctgctctttggatggcacaaggagttcttca

SEQ ID NO: 8 - DNA, 83 bp, Homo sapiens
  source 1..83: mol_type = genomic DNA
cagggggcatggattttcacaaacccgactccgtggattttagtgtcctcgtcccgctccagctccaggcccgcctccaggag

SEQ ID NO: 9 - DNA, 78 bp, Homo sapiens
  source 1..78: mol_type = genomic DNA
agcacaaacgactgcttcttgaagctctccaggtcgcccgtcaggtccagctccagggggcccggggccgagctgcac

SEQ ID NO: 10 - DNA, 63 bp, Homo sapiens
  source 1..63: mol_type = genomic DNA
gtctcttgttctttttcttgctctgatgaaacctctgctgcatcctggggctttggggcattt

SEQ ID NO: 11 - DNA, 75 bp, Homo sapiens
  source 1..75: mol_type = genomic DNA
ccaggcagccataaaatattacgtagaatagaaggatcttaaaccaactgccaccggtcctgcccagaaactcct

SEQ ID NO: 12 - DNA, 55 bp, Homo sapiens
  source 1..55: mol_type = genomic DNA
tggcgaccagcatggtgatgatcactccgcggttgggtcccttcggcacgaacca

SEQ ID NO: 13 - DNA, 71 bp, Homo sapiens
  source 1..71: mol_type = genomic DNA
agtcttttgcctgtgagcacttgttcacagccttcgggggtctcccactcacacttgggcacctctgggta

SEQ ID NO: 14 - DNA, 77 bp, Homo sapiens
  source 1..77: mol_type = genomic DNA
cgagtattttgggtagcttggaaaaatccataatgttagtttacctgctggggcgcgaggtgcagagactgtaccga

SEQ ID NO: 15 - DNA, 62 bp, Homo sapiens
  source 1..62: mol_type = genomic DNA
aggacacactccaccgcttctccctcttggccgtggactggctgcggtagcggtcgaaagtg

SEQ ID NO: 16 - DNA, 79 bp, Homo sapiens
  source 1..79: mol_type = genomic DNA
tgaaagcaaaatgtccgtagattcgtgagtttcattataataaccttctttaatgatctttcttgcaacagaaaccaaa

SEQ ID NO: 17 - DNA, 56 bp, Homo sapiens
  source 1..56: mol_type = genomic DNA
agtagcatccatcaaacagctttggcaacagctgttctctgttgagcctgcttctg

SEQ ID NO: 18 - DNA, 61 bp, Homo sapiens
  source 1..61: mol_type = genomic DNA
tcattggccaagcgctccttcaggtgctctctatcactgtagtcatctacaaggatcactt

SEQ ID NO: 19 - DNA, 71 bp, Homo sapiens
  source 1..71: mol_type = genomic DNA
ttgttcactggtcaggagccttgggacaccttttgcattatttccggacaattgctggtggccgggatccc

SEQ ID NO: 20 - DNA, 71 bp, Homo sapiens
  source 1..71: mol_type = genomic DNA
tggaacaggtggggcgttcaggagccggcattcttctctgacggcttcagatttgggaggcactggaggtg

SEQ ID NO: 21 - DNA, 57 bp, Homo sapiens
  source 1..57: mol_type = genomic DNA
ctcacacatctgtcatttagttggtcacagttgggcaggtagaagcgggttaaaagt

SEQ ID NO: 22 - DNA, 72 bp, Homo sapiens
  source 1..72: mol_type = genomic DNA
tgaactggatacagctgtcagccggcgaggccattttgtcttcaccaatgccttgcttcacagtccaaaatt

SEQ ID NO: 23 - DNA, 56 bp, Homo sapiens
  source 1..56: mol_type = genomic DNA
atgctgctgatattgacgacgcggcctttggcccttcggatgagggggagaaagga

SEQ ID NO: 24 - DNA, 71 bp, Homo sapiens
  source 1..71: mol_type = genomic DNA
tcttcagcaaccttccggtggatggagaaggactgcccaaatgcctctttgagctgctccagctcctgttt

SEQ ID NO: 25 - DNA, 75 bp, Homo sapiens
  source 1..75: mol_type = genomic DNA
gagtccaccatcacagcaaaagcatttgacatcatcactgttacccacataataaaaacccgcacttgcaagctg

SEQ ID NO: 26 - DNA, 66 bp, Homo sapiens
  source 1..66: mol_type = genomic DNA
agtgtaaaatcgaatttcatattcaaatgcccgtttctgctgctgaagagtattgttacaggcaga

SEQ ID NO: 27 - DNA, 63 bp, Homo sapiens
  source 1..63: mol_type = genomic DNA
taacctagactgacagctcacagagcaaggaggtggcagagacctgcccaggtgagcttggct

SEQ ID NO: 28 - DNA, 77 bp, Homo sapiens
  source 1..77: mol_type = genomic DNA
atagtctggaactggaggcctagaactctggttgtatttcctagaaggacagccattcatttttgcaaagagcaatc

SEQ ID NO: 29 - DNA, 63 bp, Homo sapiens
  source 1..63: mol_type = genomic DNA
ttggataagttggatgtgcttcaagaacctggtgacatatgtcaattgaatccacatatcttt

SEQ ID NO: 30 - DNA, 60 bp, Homo sapiens
  source 1..60: mol_type = genomic DNA
aggcaatgtggttgttctgcatgacctcaaagatcattcgctgaagaccaaagcagaatg

SEQ ID NO: 31 - DNA, 64 bp, Homo sapiens
  source 1..64: mol_type = genomic DNA
catgcaaattagatagagttcaatttgcagatgctaatcctcatccttgatcttgttccttcct

SEQ ID NO: 32 - DNA, 54 bp, Homo sapiens
  source 1..54: mol_type = genomic DNA
agaagccgtaggtggtgcgcacacggggcaggtgcggcagtgacagcgctgcct

SEQ ID NO: 33 - DNA, 66 bp, Homo sapiens
  source 1..66: mol_type = genomic DNA
gctttaatgtcaaagggcattggatcatcactcttgaaggcgacggccgcgttgttgaccagtacg

SEQ ID NO: 34 - DNA, 58 bp, Homo sapiens
  source 1..58: mol_type = genomic DNA
atggcctggagcgtggcttcatccttcacaaaacagaagcggatatagtggtcaaagt

SEQ ID NO: 35 - DNA, 57 bp, Homo sapiens
  source 1..57: mol_type = genomic DNA
aggtacatctgggggaaggccacagtcaccccacacggccggcaggcacaacagcac

SEQ ID NO: 36 - DNA, 72 bp, Homo sapiens
  source 1..72: mol_type = genomic DNA
cttcttttggaattttaaggccagggtttcgcttcttgcctttcgactgagacattttcccctttcctttga

SEQ ID NO: 37 - DNA, 71 bp, Homo sapiens
  source 1..71: mol_type = genomic DNA
aaagtgctctggcctcagctgcctctgtcctgtagccgtgaagcctccctcagaggcagcagaagcaacag

SEQ ID NO: 38 - DNA, 65 bp, Homo sapiens
  source 1..65: mol_type = genomic DNA
aacatcatgacagcgcccacagcgatgaggatgtagatgcctacatagaaggtgttgggcgcggg

SEQ ID NO: 39 - DNA, 68 bp, Homo sapiens
  source 1..68: mol_type = genomic DNA
aacctggaatcctgcataagcacatcctgaagactgactatatttggatgacgaagttcctttaatag

SEQ ID NO: 40 - DNA, 63 bp, Homo sapiens
  source 1..63: mol_type = genomic DNA
atgagttgaagcagtttggagccacagtctgtgataaacggagtgtattggttttgctttcaa

SEQ ID NO: 41 - DNA, 57 bp, Homo sapiens
  source 1..57: mol_type = genomic DNA
gggaggggttaataaggcaacagttaaaaacggtccattttatcaaaaccgacacct

SEQ ID NO: 42 - DNA, 60 bp, Homo sapiens
  source 1..60: mol_type = genomic DNA
tcggggacaggttgagcagttatatggctctggcagaggggcgggggcagagggaggggt

SEQ ID NO: 43 - DNA, 60 bp, Homo sapiens
  source 1..60: mol_type = genomic DNA
aatcattagccggagcacggtgtacttgcgcatcagcttctttacttcccgatcttcttc

SEQ ID NO: 44 - DNA, 73 bp, Homo sapiens
  source 1..73: mol_type = genomic DNA
ccgtaggtgcaaaagcaacatccacatctcactcctcccggtgctttttgcggtattcctgcagcgctttctc

SEQ ID NO: 45 - DNA, 66 bp, Homo sapiens
  source 1..66: mol_type = genomic DNA
caatttgagtccttcctgctgtgaaggtgggcattgtgcacctgtatttgccccatggccgaaggt

SEQ ID NO: 46 - DNA, 64 bp, Homo sapiens
  source 1..64: mol_type = genomic DNA
caagaacttcacaatattacccacagcctcttcaagtgtcttgatggtagacaaggtgaacgtt

SEQ ID NO: 47 - DNA, 65 bp, Homo sapiens
  source 1..65: mol_type = genomic DNA
cacagcaatcttcctcagcatcacattcacccccagcactttgagcaattcctcgaagttttccg

SEQ ID NO: 48 - DNA, 61 bp, Homo sapiens
  source 1..61: mol_type = genomic DNA
tggctgggactttcagattgacttgaatctgctgcatgcacaaagtatgccaaatataaat

SEQ ID NO: 49 - DNA, 77 bp, Homo sapiens
  source 1..77: mol_type = genomic DNA
cacttgtgtttgggtggttaacaaagcagtaaaagcgggatccttatcttcatttgctggaaaagatggaagcagcc

SEQ ID NO: 50 - DNA, 79 bp, Homo sapiens
  source 1..79: mol_type = genomic DNA
gctttctgcagacatactatggactcctccgccagcacctcacttctcctcatggcggacgctccaagcagccgtgagt

SEQ ID NO: 51 - DNA, 59 bp, Homo sapiens
  source 1..59: mol_type = genomic DNA
acttgtttccacctccccagacaggcattttgagtcggaggcgggagcacgtaccgcag

SEQ ID NO: 52 - DNA, 76 bp, Homo sapiens
  source 1..76: mol_type = genomic DNA
ttcactctcgtggtggtcacaatgcccacagatttcccagcgtccttggcccagcgcaggatggaggtgacctcgt

SEQ ID NO: 53 - DNA, 76 bp, Homo sapiens
  source 1..76: mol_type = genomic DNA
actcagtgtctgccatgtcatcaaaccaggactgcacaggcactgcattctcggggtggaatatgtaagaagcagg

SEQ ID NO: 54 - DNA, 55 bp, Homo sapiens
  source 1..55: mol_type = genomic DNA
ttcagctctagcggctggggacctaggtcctgggccctaagggggcctctgatgc

SEQ ID NO: 55 - DNA, 62 bp, Homo sapiens
  source 1..62: mol_type = genomic DNA
ctcaagcttgtgtaatagacctccagaacaccttggactggagagaggctgctgaccagcag

SEQ ID NO: 56 - DNA, 77 bp, Homo sapiens
  source 1..77: mol_type = genomic DNA
aaaacaccttctggcgggaatgtactgtatgcaggatctctcagggaaaaaatcagtttctctgtcaatcccataag

SEQ ID NO: 57 - DNA, 77 bp, Homo sapiens
  source 1..77: mol_type = genomic DNA
ttctttgctccttccatgcctggccacttgacataatcaatccatttttcttaaagatatgttctcgcataggggtc

SEQ ID NO: 58 - DNA, 62 bp, Homo sapiens
  source 1..62: mol_type = genomic DNA
gcactctgtgtcaaatttccagagaccctgacgataggacaaaacatttcccaacaaaggca

SEQ ID NO: 59 - DNA, 70 bp, Homo sapiens
  source 1..70: mol_type = genomic DNA
gggatcaggtttcatcaaggactttatctctggatactttgccaggatctcccggcgccggtcggcgtgc

SEQ ID NO: 60 - DNA, 79 bp, Homo sapiens
  source 1..79: mol_type = genomic DNA
agtcattcagctgcacatgtatggtgtagtcctcattccggaacttgggatttgaactgttccagaagacggtgtggcg

SEQ ID NO: 61 - DNA, 70 bp, Homo sapiens
  source 1..70: mol_type = genomic DNA
cgcttctccgccagcgtcagcgccttccacgacttgcccagcatcttgctcaactcggcgttgtgcaggt

SEQ ID NO: 62 - DNA, 67 bp, Homo sapiens
  source 1..67: mol_type = genomic DNA
tgttgccaggacattggactgccagggacaccatgctacggccttgacagccccttgatgctgggtg

SEQ ID NO: 63 - DNA, 63 bp, Homo sapiens
  source 1..63: mol_type = genomic DNA
actcctcgtcctctgcgcacgggtacggctggtagttgtcaatggtctggtacttattcccgc

SEQ ID NO: 64 - DNA, 71 bp, Homo sapiens
  source 1..71: mol_type = genomic DNA
agagcacagatcgggacagcagccctggaagccgtcgaagcctcctcgcaggaagtacacggcagtgggcc

SEQ ID NO: 65 - DNA, 57 bp, Homo sapiens
  source 1..57: mol_type = genomic DNA
cttcctcagcattgaagccaacctcgtcgcagtggcgatggtactcctccatggtag

SEQ ID NO: 66 - DNA, 57 bp, Homo sapiens
  source 1..57: mol_type = genomic DNA
tctgcgatgatgtactcaaagttagcacccgaggcgaagggacgccaggcgggacag

SEQ ID NO: 67 - DNA, 60 bp, Homo sapiens
  source 1..60: mol_type = genomic DNA
gcatgttacaaggtccttcagtggcctgcttatatagcgcgtagagttttagcttcactt

SEQ ID NO: 68 - DNA, 62 bp, Homo sapiens
  source 1..62: mol_type = genomic DNA
ttggacagtccatagggcaccgtctgttcgggagtgttgatccaaatgatgtccaggtggca

SEQ ID NO: 69 - DNA, 75 bp, Homo sapiens
  source 1..75: mol_type = genomic DNA
tcaaaagttgttcgagtccatttatcatccactgactcttctttcgccactggcatatttgaaagtgctccgtat

SEQ ID NO: 70 - DNA, 78 bp, Homo sapiens
  source 1..78: mol_type = genomic DNA
gggccagagccgatgtcaatcagcaggtctcccttcacaccgtctaggcagaatatcttgaaaagatttttcagaagg

SEQ ID NO: 71 - DNA, 71 bp, Homo sapiens
  source 1..71: mol_type = genomic DNA
cattcaattaatttagctctcagcaactctttgaggcgttctctttctccagtttctatcaacttttggtt

SEQ ID NO: 72 - DNA, 56 bp, Homo sapiens
  source 1..56: mol_type = genomic DNA
tacccattttgtgtccatgagggtctcttccagcgcccggcagccggcgggcagca

SEQ ID NO: 73 - DNA, 76 bp, Homo sapiens
  source 1..76: mol_type = genomic DNA
tccacctttggagtctttccttctgattcacgattttctttcaacaattttccacttaggaatccatcacaaaagt

SEQ ID NO: 74 - DNA, 71 bp, Homo sapiens
  source 1..71: mol_type = genomic DNA
gggcaggggcttcttccttttagtccttaggggcttctctagcagcccacgcttagcaggcaacagtttgc

SEQ ID NO: 75 - DNA, 56 bp, Homo sapiens
  source 1..56: mol_type = genomic DNA
agacgctttggtgaagtatccagcaaccctgtacagataaagccagggagccctcc

SEQ ID NO: 76 - DNA, 77 bp, Homo sapiens
  source 1..77: mol_type = genomic DNA
tccagttctgaggagtactcattgactacattttcattatcttttacttgcttctgcctcttttgccacaggtcttt

SEQ ID NO: 77 - DNA, 64 bp, Homo sapiens
  source 1..64: mol_type = genomic DNA
agccaggcatatctacccggaatttctgctggccgccgccgccgctggagtaggactcggcgtg

SEQ ID NO: 78 - DNA, 67 bp, Homo sapiens
  source 1..67: mol_type = genomic DNA
ctcttgaagttcttggtcacaaactcctgcagtgcttcagtccaaagcagaggagtcttgaatcagg

SEQ ID NO: 79 - DNA, 65 bp, Homo sapiens
  source 1..65: mol_type = genomic DNA
gtgtagggacagattatgacgaattgaattcttccagcccgccgagctgttgctgtcacccttat

SEQ ID NO: 80 - DNA, 75 bp, Homo sapiens
  source 1..75: mol_type = genomic DNA
acttctttccagagctgctgcagttctgttggaatcatgccttgagcaagaggttgaaggggaagggcaggctgc

SEQ ID NO: 81 - DNA, 72 bp, Homo sapiens
  source 1..72: mol_type = genomic DNA
agatcaggcaccctggcttttggagccttctctacaatcacggggaccctgtccggatatttcttccggatc

SEQ ID NO: 82 - DNA, 60 bp, Homo sapiens
  source 1..60: mol_type = genomic DNA
cagtgttggaaatgtcatgacaatgcagtgctgcacagcagcaaaactcaatcccaaact

SEQ ID NO: 83 - DNA, 62 bp, Homo sapiens
  source 1..62: mol_type = genomic DNA
aatttgggctagtgctgggtcccaagtcatgtatagcatatcactggctgttggtttcacct

SEQ ID NO: 84 - DNA, 69 bp, Homo sapiens
  source 1..69: mol_type = genomic DNA
caaaaccttgaattctttcatatgcttttttaagttgaatttcaattccatttgcatatttggagtata

SEQ ID NO: 85 - DNA, 57 bp, Homo sapiens
  source 1..57: mol_type = genomic DNA
acaagcacactcggggctgctggccaggccgtgtgcgcagagcagggcgccaagcag

SEQ ID NO: 86 - DNA, 79 bp, Homo sapiens
  source 1..79: mol_type = genomic DNA
ccgtactcgtaaatggtgccacttatgccaccatggcagtccatcttcgacttctcttgtccccggctctgcgagacga

SEQ ID NO: 87 - DNA, 76 bp, Homo sapiens
  source 1..76: mol_type = genomic DNA
tgtgaggccttgtaggtttccaaacattcttccattaatagcatgcattttattgctttctatgaattcctcatca

SEQ ID NO: 88 - DNA, 57 bp, Homo sapiens
  source 1..57: mol_type = genomic DNA
tctcatcctggctgcactcattgcccagccagtagtggaggtcatactgcagatttc

SEQ ID NO: 89 - DNA, 63 bp, Homo sapiens
  source 1..63: mol_type = genomic DNA
taagagggtcattttgggccttcacatccctctcgggcctcaagttcccgtcgcggcgtcccc

SEQ ID NO: 90 - DNA, 63 bp, Homo sapiens
  source 1..63: mol_type = genomic DNA
caatgtaagagatacgttggaccctcttctctcttgaagtcctatgggcttcattttgaaagg

SEQ ID NO: 91 - DNA, 70 bp, Homo sapiens
  source 1..70: mol_type = genomic DNA
ctttggatccatctttgccctctgtattctctggagactttctcttcggcataatgactatgtcggtgaa

SEQ ID NO: 92 - DNA, 62 bp, Homo sapiens
  source 1..62: mol_type = genomic DNA
actctcttgggttccttgagcccgtgtctctctgtgaccatagccagggcagcaatgcagga

SEQ ID NO: 93 - DNA, 59 bp, Homo sapiens
  source 1..59: mol_type = genomic DNA
atcaatccccagcagtggaataaggcctgttgttccttgcagtggatcctgatttggac

SEQ ID NO: 94 - DNA, 83 bp, Homo sapiens
  source 1..83: mol_type = genomic DNA
ctttgaagcacaataaaccggctgctgtgcaacgggcatgagtcctgctaaagatgacatattgataatgatgccgccttcac

SEQ ID NO: 95 - DNA, 73 bp, Homo sapiens
  source 1..73: mol_type = genomic DNA
ccaagagtcgtctagttcttcatgagaaaagcctgttaaactttcgactttgtcactagattgcagcgtgtcc

SEQ ID NO: 96 - DNA, 62 bp, Homo sapiens
  source 1..62: mol_type = genomic DNA
tatccaacacttcgtggggtccttttcaccagcaagcttgcgaccttgaccatctttggatt

SEQ ID NO: 97 - DNA, 62 bp, Homo sapiens
  source 1..62: mol_type = genomic DNA
aaaagtagcccacccgggtgtcctagtcactcccttcggagctccgactaagcccgatcgcg

SEQ ID NO: 98 - DNA, 71 bp, Homo sapiens
  source 1..71: mol_type = genomic DNA
ttcctcccagtcttgcagactcaactgaatgtagtttatcgcctgccgggatgatatgctggcgaagagtt

SEQ ID NO: 99 - DNA, 75 bp, Homo sapiens
  source 1..75: mol_type = genomic DNA
agagttccattatccgctacatctgaatgacctgcattaaaatatttcttaaggttttctgcttcttttacatat

SEQ ID NO: 100 - DNA, 72 bp, Homo sapiens
  source 1..72: mol_type = genomic DNA
agcatcgacttccccattgggattcccattggtgtctggaagccggcgacgctgccgcccacctccctgctg

SEQ ID NO: 101 - DNA, 76 bp, Homo sapiens
  source 1..76: mol_type = genomic DNA
tccagttcctcacattctttgcatccagattctgttacattcccattagaagacaaactgttgtttgctaggatga

SEQ ID NO: 102 - DNA, 73 bp, Homo sapiens
  source 1..73: mol_type = genomic DNA
ttctcttatggcagcgggaccatgctccactccttttcttttctgcccttgtgagaacggggctcctatcaca

SEQ ID NO: 103 - DNA, 79 bp, Homo sapiens
  source 1..79: mol_type = genomic DNA
tggtgttggctttgggcgcccccaccaagacactcgctgtgcgggcgtcgggtatgtggaagtccacggcgtagccgaa

SEQ ID NO: 104 - DNA, 59 bp, Homo sapiens
  source 1..59: mol_type = genomic DNA
agattgtgcagggcctcgaagaccaccgtcacctcttctgggttcccatgagctatttc

SEQ ID NO: 105 - DNA, 61 bp, Homo sapiens
  source 1..61: mol_type = genomic DNA
ctcctttggaacccagtctcgaaaacctagaggaggtccatgtgtcatgagtatgtcaatg

SEQ ID NO: 106 - DNA, 58 bp, Homo sapiens
  source 1..58: mol_type = genomic DNA
tgactcagctgacatccagagaacatgtcctgttgctggcgcaggagcatggggacat

SEQ ID NO: 107 - DNA, 77 bp, Homo sapiens
  source 1..77: mol_type = genomic DNA
agttaatgcttcttccacgtgtgaaggtagccactcgagtatcttccctagcttcatatacatcaatctggaaattc

SEQ ID NO: 108 - DNA, 67 bp, Homo sapiens
  source 1..67: mol_type = genomic DNA
tcagcacgtagttggggtccaggtcgtcgccgccctgcaggttgtcggggttgaggtcggtcttgtg

SEQ ID NO: 109 - DNA, 74 bp, Homo sapiens
  source 1..74: mol_type = genomic DNA
tgttctgggccgtcatttgtgatttggcctggagtgtaggttcttcagaagaagtgatgggtcctttaggtaat

SEQ ID NO: 110 - DNA, 57 bp, Homo sapiens
  source 1..57: mol_type = genomic DNA
tcaggatctgcatacacctgcccaatgatctcacagagaacgatcccaaaggagaag

SEQ ID NO: 111 - DNA, 72 bp, Homo sapiens
  source 1..72: mol_type = genomic DNA
acacctcttgctgactgcagctggcccagggacatctttttaactcctgggttgaggtccttagccaccttt

SEQ ID NO: 112 - DNA, 72 bp, Homo sapiens
  source 1..72: mol_type = genomic DNA
atatctggagggatgttgtttggcacttttttcaactctttccttttgcagtccagtgtttgtatgggaaac

SEQ ID NO: 113 - DNA, 57 bp, Homo sapiens
  source 1..57: mol_type = genomic DNA
taagggaaccgcaggatggccatctcaatcatggtgatgcccaggctccagacgtcg

SEQ ID NO: 114 - DNA, 56 bp, Homo sapiens
  source 1..56: mol_type = genomic DNA
tcctccgtctcgtcgtcctctccgtctccaatgcggaagtcgatgtagccctcccc

SEQ ID NO: 115 - DNA, 65 bp, Homo sapiens
  source 1..65: mol_type = genomic DNA
aaatgttggttgctgtcttcatctttgtgtatcggatgatcacgaacatgaccagcgagttgccc

SEQ ID NO: 116 - DNA, 56 bp, Homo sapiens
  source 1..56: mol_type = genomic DNA
gtgcacgggtactgttcctcacggcagtcaagaggcccaggctctgtgggctccag

SEQ ID NO: 117 - DNA, 59 bp, Homo sapiens
  source 1..59: mol_type = genomic DNA
ttctcacaggtcagggggcctccagagtcaccctggcaggtgtcttgcccaggtttctg

SEQ ID NO: 118 - DNA, 54 bp, Homo sapiens
  source 1..54: mol_type = genomic DNA
cagccatctgacggcaaagctcatctttcatagcttcgtgttccttacagacaa

SEQ ID NO: 119 - DNA, 63 bp, Homo sapiens
  source 1..63: mol_type = genomic DNA
cgaaattgctgcagtcaaatggtgatttcactttcggccggaacggtgggtcaatctccttcc

SEQ ID NO: 120 - DNA, 67 bp, Homo sapiens
  source 1..67: mol_type = genomic DNA
ggagggatacaaggaaggtttcagaatccaagccggcggcggcggggctccggcaggatcgcgaaca

SEQ ID NO: 121 - DNA, 54 bp, Homo sapiens
  source 1..54: mol_type = genomic DNA
cacctgcatggtcaagatagacagttcctgccaggcggctgaactcgcgcgccc

SEQ ID NO: 122 - DNA, 77 bp, Homo sapiens
  source 1..77: mol_type = genomic DNA
ggcttgacatctttatggtggtcactagcgttccatcagttgtttcaaccaaggaggtcttggcaggaactgaaata

SEQ ID NO: 123 - DNA, 73 bp, Homo sapiens
  source 1..73: mol_type = genomic DNA
atactcatcacttggcacccgtcttggaagaggggaacccgtagctccccgccgaccccgatggtcccctccc

SEQ ID NO: 124 - DNA, 72 bp, Homo sapiens
  source 1..72: mol_type = genomic DNA
agggggtcagtagccagcaccgtcaagttcccagccgaatacagttctttaagctggtcgtggttaccctgc

SEQ ID NO: 125 - DNA, 79 bp, Homo sapiens
  source 1..79: mol_type = genomic DNA
aaactggtgttcccttgattcagggccagtgtgaacaccatttcccactggtccaaatgtacctgtacccatattacta

SEQ ID NO: 126 - DNA, 76 bp, Homo sapiens
  source 1..76: mol_type = genomic DNA
aggtcccacggtcatccacggagccggtgaaattggaaaacaactgggacacagaacctccgctgcctaagctgcg

SEQ ID NO: 127 - DNA, 74 bp, unidentified
  source 1..74: mol_type = genomic DNA
tctccaaggaccttcttctcaacacagctgttgttctcccatctgtgcagaacgatctccaggttgtcctcggg

SEQ ID NO: 128 - DNA, 66 bp, Homo sapiens
  source 1..66: mol_type = genomic DNA
aatcaggtctccaggcttaggctctggaatgggcgcacgcatcttccctcgcggtgtggaccctca

SEQ ID NO: 129 - DNA, 71 bp, Homo sapiens
  source 1..71: mol_type = genomic DNA
cctgatcacacagagccatactaaatcgtaggtctgggcatgagcaaacttcaagagacatttctagaacc

SEQ ID NO: 130 - DNA, 56 bp, Homo sapiens
  source 1..56: mol_type = genomic DNA
cgaggcggggcgtagacctgcggctctgggattccgttgcctgacactgtgctctc

SEQ ID NO: 131 - DNA, 65 bp, Homo sapiens
  source 1..65: mol_type = genomic DNA
gcagtgttcttataatcttcataggtgtatccgttctccatggtctcgcagacgccttctcgatg

SEQ ID NO: 132 - DNA, 71 bp, Homo sapiens
  source 1..71: mol_type = genomic DNA
tctttttggtgcccaaaatctgttgaagggcacagacatttgggccttggtcccgacccctgatacgacta

SEQ ID NO: 133 - DNA, 71 bp, Homo sapiens
  source 1..71: mol_type = genomic DNA
aaggacaggtgtggtgcttgcgtttcctgaagaaggggaccttgtggctgccggggtggcactcctcgcct

SEQ ID NO: 134 - DNA, 61 bp, Homo sapiens
  source 1..61: mol_type = genomic DNA
cagaggactacactggtctggaatggcattgacacagcttcttaggtcaggataagcatta

SEQ ID NO: 135 - DNA, 75 bp, Homo sapiens
  source 1..75: mol_type = genomic DNA
tgtcgctcgctgatatgctcttcaatttcaaacacttctccagaggttatattaatatttccagcttcgatccct

SEQ ID NO: 136 - DNA, 54 bp, Homo sapiens
  source 1..54: mol_type = genomic DNA
tctggccaaggtacgaagctttggagaacccaggaggatgaggaaccgcgggtc

SEQ ID NO: 137 - DNA, 58 bp, Homo sapiens
  source 1..58: mol_type = genomic DNA
agtggctaccggggtgtggtcagctgctgtccctttggtttttgtagccgagcagggg

SEQ ID NO: 138 - DNA, 56 bp, Homo sapiens
  source 1..56: mol_type = genomic DNA
cgggaggacgcgttccaatgatgcatttctttggcagttctcgaaggagaagcccc

SEQ ID NO: 139 - DNA, 85 bp, Homo sapiens
  source 1..85: mol_type = genomic DNA
caggtaagggttaatctcaatcaccttgttcacccgtaaggcactaatgtaggacccagctgaggcccgagaatccactgctgca

SEQ ID NO: 140 - DNA, 68 bp, Homo sapiens
  source 1..68: mol_type = genomic DNA
ggagctagccattatcttgtgggcagccaagacgcctgctgctgtgaagcccttggccagggcaaaag

SEQ ID NO: 141 - DNA, 64 bp, Homo sapiens
  source 1..64: mol_type = genomic DNA
agcaggatggtggtcgtcttgtagtcgatgcccgccgggtggccgtacggggactcggccgcgc

SEQ ID NO: 142 - DNA, 69 bp, Homo sapiens
  source 1..69: mol_type = genomic DNA
atcctcaaagtccttcgccaactggataaattggacttcatttccttcactgagaatctccacccggcg

SEQ ID NO: 143 - DNA, 66 bp, Homo sapiens
  source 1..66: mol_type = genomic DNA
aatcaggtctccaggtttgggctcttggtgtggcgaagccatctcgaagccaagaggaggtctggt

SEQ ID NO: 144 - DNA, 75 bp, Homo sapiens
  source 1..75: mol_type = genomic DNA
ttaattttggacagctggcacatccaaatgctatcacagcatatccacagtctggagctggacaccacctacaat

SEQ ID NO: 145 - DNA, 59 bp, Homo sapiens
  source 1..59: mol_type = genomic DNA
cagtcacgagctacgagttctattctgggtctttgtcccagggccagcaggaacgctag

SEQ ID NO: 146 - DNA, 64 bp, Homo sapiens
  source 1..64: mol_type = genomic DNA
atcagcttctggaaagcagcttcatctgtccttttccccaagaagctgggcagctcccgggtca

SEQ ID NO: 147 - DNA, 74 bp, Homo sapiens
  source 1..74: mol_type = genomic DNA
gaaaaagttttctagctctttaccttcaatatacccatttccgtctgcgtcaaagtgcttccatatttccagga

SEQ ID NO: 148 - DNA, 72 bp, Homo sapiens
  source 1..72: mol_type = genomic DNA
ggaacatttcttgtcacttgtgtaactgatggatccttgaagggattgttgagatccgggtcggcaaacggg

SEQ ID NO: 149 - DNA, 65 bp, Homo sapiens
  source 1..65: mol_type = genomic DNA
atcacaaagactgctgtcatatattaattgcataaacacctcaacattgctcagagtttcatccg

SEQ ID NO: 150 - DNA, 57 bp, Homo sapiens
  source 1..57: mol_type = genomic DNA
tcggctcagccaaacactgtcagggcccccagcagggccttcagggccttcacggcc

SEQ ID NO: 151 - DNA, 66 bp, Homo sapiens
  source 1..66: mol_type = genomic DNA
gatgtgggctcgttcctcaaaaattgagatggttttatggctacagctgctgagtggtgggtgaaa

SEQ ID NO: 152 - DNA, 74 bp, Homo sapiens
  source 1..74: mol_type = genomic DNA
ctgtaccatcatgtctggtgtgatgtctatccacttaacatcctccgggaggtccgtgacgatggcttcaggcg

SEQ ID NO: 153 - DNA, 76 bp, Homo sapiens
  source 1..76: mol_type = genomic DNA
cccagctgatgaaatttgtgaagtacagaatcaggattgctcgcattccatagtaggaaaatctttcgcaaaactc

SEQ ID NO: 154 - DNA, 68 bp, Homo sapiens
  source 1..68: mol_type = genomic DNA
aaacgattgctcaggactgtggcgaggggagctgaaaatgttaagacaaacacacagattgagattat

SEQ ID NO: 155 - DNA, 76 bp, Homo sapiens
  source 1..76: mol_type = genomic DNA
caagatgctgaacgctggcaaaaatggtaagaatggaaccatgaaggctactttttgctgattctggggctgcctc

SEQ ID NO: 156 - DNA, 68 bp, Homo sapiens
  source 1..68: mol_type = genomic DNA
cacttctgcacattgctggggctccagtccatgggatctgcggtgatgttgagcagcttgcaggccgt

SEQ ID NO: 157 - DNA, 58 bp, Homo sapiens
  source 1..58: mol_type = genomic DNA
ttaggaggacagactccagctttgaaggactttccagagccttccacagcccaaggtg

SEQ ID NO: 158 - DNA, 80 bp, Homo sapiens
  source 1..80: mol_type = genomic DNA
gaaggctgctatctgaaagcaaaagtgcattctgtaggacttttctgaggaaatcttccagaccctggcgacgctgatcc

SEQ ID NO: 159 - DNA, 71 bp, Homo sapiens
  source 1..71: mol_type = genomic DNA
ctccccaggttatagtcatagagctttgtcaaaatgagaatcacgctgctgttgtggccagaccagtggac

SEQ ID NO: 160 - DNA, 76 bp, Homo sapiens
  source 1..76: mol_type = genomic DNA
tttccatgtgtgaggtgatgtcctcgtctgtagcatcagggtactggatgtcaggtctgcgaaacttcttagattt

SEQ ID NO: 161 - DNA, 69 bp, Homo sapiens
  source 1..69: mol_type = genomic DNA
tcctattaagcttgtttctgaaatattggttccttttctgcgcctcctggcctcgagctgctccttatt

SEQ ID NO: 162 - DNA, 59 bp, Homo sapiens
  source 1..59: mol_type = genomic DNA
ttgatgatgctcttgggcagccaccccttgaggtcgatgctgagtagccacgtaagttt

SEQ ID NO: 163 - DNA, 67 bp, Homo sapiens
  source 1..67: mol_type = genomic DNA
gacctgtagagcactgttgaggcaacgaaccacttcagctgagttttgagccgccactcgggatttc

SEQ ID NO: 164 - DNA, 59 bp, Homo sapiens
  source 1..59: mol_type = genomic DNA
agagggtcgaaggtgaagatctcaggaccggagccccgccggggtcccgggatggtgga

SEQ ID NO: 165 - DNA, 59 bp, Homo sapiens
  source 1..59: mol_type = genomic DNA
agggcgccagggcgctctccttggcccccggcttcctgtggtcggccatgagcgcctcc

SEQ ID NO: 166 - DNA, 59 bp, Homo sapiens
  source 1..59: mol_type = genomic DNA
aactcttgcaggtaccagagcttacctgaggccatctcagacaaaagtaagcagagagt

SEQ ID NO: 167 - DNA, 74 bp, Homo sapiens
  source 1..74: mol_type = genomic DNA
tgggctgtacacaagatcagggtcaaataacccagtttggactggacaaatcggaactctctccagttgactgc

SEQ ID NO: 168 - DNA, 60 bp, Homo sapiens
  source 1..60: mol_type = genomic DNA
tatgatcatgcccatggctgtctctagttccgtcatggtgctagattcagacccaccttc

SEQ ID NO: 169 - DNA, 73 bp, Homo sapiens
  source 1..73: mol_type = genomic DNA
atccgtgcctggaggtaatagtagctttccatagggtggtttataaggggtgctggacgcagggggaacaggt

SEQ ID NO: 170 - DNA, 79 bp, Homo sapiens
  source 1..79: mol_type = genomic DNA
agtccaccctgtccttggctggcacggcacactggtttgcagacaggcccacgtactcctcagcagagctggaggacag

SEQ ID NO: 171 - DNA, 72 bp, Homo sapiens
  source 1..72: mol_type = genomic DNA
ttcacggagaaggggcgctggatgcgtgaggcatagctcctgagcttgtccttggcgtcactgaagctctca

SEQ ID NO: 172 - DNA, 73 bp, Homo sapiens
  source 1..73: mol_type = genomic DNA
gccccatcttcaattgtctggatttcacacctggataaatccagcacctgcagttctgggaaactgaagaagc

SEQ ID NO: 173 - DNA, 74 bp, Homo sapiens
  source 1..74: mol_type = genomic DNA
tctggagcaacttgcctgcagagatttctgtatccacggacatttaaatatcgcaaaggctatctccaggcaag

SEQ ID NO: 174 - DNA, 55 bp, Homo sapiens
  source 1..55: mol_type = genomic DNA
tgtttgtcaggcgggagcctggagcctgcacagggacagagctggtttcatccgg

SEQ ID NO: 175 - DNA, 66 bp, Homo sapiens
  source 1..66: mol_type = genomic DNA
ctcttccacatatgtggatggaaaccagcccaccctgccatttacttctcctctccaccagccatt

SEQ ID NO: 176 - DNA, 59 bp, Homo sapiens
  source 1..59: mol_type = genomic DNA
agacgcccataagagaagcgcgccggctgagggtgcaggagaggcgagagcgcgccccg

SEQ ID NO: 177 - DNA, 75 bp, Homo sapiens
  source 1..75: mol_type = genomic DNA
gctcataatcactggcttccatgtcttcaccacaggaatcattccaatacgttctctttctacgacgacactgtc

SEQ ID NO: 178 - DNA, 60 bp, Homo sapiens
  source 1..60: mol_type = genomic DNA
ctctggatctgcatttttctccaccacctttctgccattcacaaagaaaaccaatttgtc

SEQ ID NO: 179 - DNA, 27 bp, Homo sapiens
  source 1..27: mol_type = genomic DNA
ggacgccctgtgcggttccggggagct

SEQ ID NO: 180 - DNA, 27 bp, Homo sapiens
  source 1..27: mol_type = genomic DNA
tacttccctcctgggatcatgactcaa

SEQ ID NO: 181 - DNA, 27 bp, Homo sapiens
  source 1..27: mol_type = genomic DNA
tctgaacgagtcggacttcctcaacaa

SEQ ID NO: 182 - DNA, 29 bp, Homo sapiens
  source 1..29: mol_type = genomic DNA
gacccggcctgggagaagcagcagagaaa

SEQ ID NO: 183 - DNA, 22 bp, Homo sapiens
  source 1..22: mol_type = genomic DNA
tccgcaacctggaggtcaagtt

SEQ ID NO: 184 - DNA, 29 bp, Homo sapiens
  source 1..29: mol_type = genomic DNA
aagtttctggattcactgaatcaacagac

SEQ ID NO: 185 - DNA, 26 bp, Homo sapiens
  source 1..26: mol_type = genomic DNA
tgaagaactccttgtgccatccaaag

SEQ ID NO: 186 - DNA, 26 bp, Homo sapiens
  source 1..26: mol_type = genomic DNA
ctcctggaggcgggcctggagctgga

SEQ ID NO: 187 - DNA, 30 bp, Homo sapiens
  source 1..30: mol_type = genomic DNA
gtgcagctcggccccgggccccctggagct

SEQ ID NO: 188 - DNA, 22 bp, Homo sapiens
  source 1..22: mol_type = genomic DNA
aaatgccccaaagccccaggat

SEQ ID NO: 189 - DNA, 23 bp, Homo sapiens
  source 1..23: mol_type = genomic DNA
aggagtttctgggcaggaccggt

SEQ ID NO: 190 - DNA, 23 bp, Homo sapiens
  source 1..23: mol_type = genomic DNA
tggttcgtgccgaagggacccaa

SEQ ID NO: 191 - DNA, 25 bp, Homo sapiens
  source 1..25: mol_type = genomic DNA
tacccagaggtgcccaagtgtgagt

SEQ ID NO: 192 - DNA, 22 bp, Homo sapiens
  source 1..22: mol_type = genomic DNA
tcggtacagtctctgcacctcg

SEQ ID NO: 193 - DNA, 26 bp, Homo sapiens
  source 1..26: mol_type = genomic DNA
cactttcgaccgctaccgcagccagt

SEQ ID NO: 194 - DNA, 27 bp, Homo sapiens
  source 1..27: mol_type = genomic DNA
tttggtttctgttgcaagaaagatcat

SEQ ID NO: 195 - DNA, 24 bp, Homo sapiens
  source 1..24: mol_type = genomic DNA
cagaagcaggctcaacagagaaca

SEQ ID NO: 196 - DNA, 27 bp, Homo sapiens
  source 1..27: mol_type = genomic DNA
aagtgatccttgtagatgactacagtg

SEQ ID NO: 197 - DNA, 24 bp, Homo sapiens
  source 1..24: mol_type = genomic DNA
gggatcccggccaccagcaattgt

SEQ ID NO: 198 - DNA, 26 bp, Homo sapiens
  source 1..26: mol_type = genomic DNA
cacctccagtgcctcccaaatctgaa

SEQ ID NO: 199 - DNA, 27 bp, Homo sapiens
  source 1..27: mol_type = genomic DNA
acttttaacccgcttctacctgcccaa

SEQ ID NO: 200 - DNA, 27 bp, Homo sapiens
  source 1..27: mol_type = genomic DNA
aattttggactgtgaagcaaggcattg

SEQ ID NO: 201 - DNA, 23 bp, Homo sapiens
  source 1..23: mol_type = genomic DNA
tcctttctccccctcatccgaag

SEQ ID NO: 202 - DNA, 24 bp, Homo sapiens
  source 1..24: mol_type = genomic DNA
aaacaggagctggagcagctcaaa

SEQ ID NO: 203 - DNA, 24 bp, Homo sapiens
  source 1..24: mol_type = genomic DNA
cagcttgcaagtgcgggtttttat

SEQ ID NO: 204 - DNA, 27 bp, Homo sapiens
  source 1..27: mol_type = genomic DNA
tctgcctgtaacaatactcttcagcag

SEQ ID NO: 205 - DNA, 26 bp, Homo sapiens
  source 1..26: mol_type = genomic DNA
agccaagctcacctgggcaggtctct

SEQ ID NO: 206 - DNA, 28 bp, Homo sapiens
  source 1..28: mol_type = genomic DNA
gattgctctttgcaaaaatgaatggctg

SEQ ID NO: 207 - DNA, 30 bp, Homo sapiens
  source 1..30: mol_type = genomic DNA
aaagatatgtggattcaattgacatatgtc

SEQ ID NO: 208 - DNA, 26 bp, Homo sapiens
  source 1..26: mol_type = genomic DNA
cattctgctttggtcttcagcgaatg

SEQ ID NO: 209 - DNA, 26 bp, Homo sapiens
  source 1..26: mol_type = genomic DNA
aggaaggaacaagatcaaggatgagg

SEQ ID NO: 210 - DNA, 22 bp, Homo sapiens
  source 1..22: mol_type = genomic DNA
aggcagcgctgtcactgccgca

SEQ ID NO: 211 - DNA, 22 bp, Homo sapiens
  source 1..22: mol_type = genomic DNA
cgtactggtcaacaacgcggcc

SEQ ID NO: 212 - DNA, 27 bp, Homo sapiens
  source 1..27: mol_type = genomic DNA
actttgaccactatatccgcttctgtt

SEQ ID NO: 213 - DNA, 25 bp, Homo sapiens
  source 1..25: mol_type = genomic DNA
gtgctgttgtgcctgccggccgtgt

SEQ ID NO: 214 - DNA, 28 bp, Homo sapiens
  source 1..28: mol_type = genomic DNA
tcaaaggaaaggggaaaatgtctcagtc

SEQ ID NO: 215 - DNA, 22 bp, Homo sapiens
  source 1..22: mol_type = genomic DNA
ctgttgcttctgctgcctctga

SEQ ID NO: 216 - DNA, 24 bp, Homo sapiens
  source 1..24: mol_type = genomic DNA
cccgcgcccaacaccttctatgta

SEQ ID NO: 217 - DNA, 29 bp, Homo sapiens
  source 1..29: mol_type = genomic DNA
ctattaaaggaacttcgtcatccaaatat

SEQ ID NO: 218 - DNA, 27 bp, Homo sapiens
  source 1..27: mol_type = genomic DNA
ttgaaagcaaaaccaatacactccgtt

SEQ ID NO: 219 - DNA, 27 bp, Homo sapiens
  source 1..27: mol_type = genomic DNA
aggtgtcggttttgataaaatggaccg

SEQ ID NO: 220 - DNA, 26 bp, Homo sapiens
  source 1..26: mol_type = genomic DNA
acccctccctctgcccccgcccctct

SEQ ID NO: 221 - DNA, 27 bp, Homo sapiens
  source 1..27: mol_type = genomic DNA
gaagaagatcgggaagtaaagaagctg

SEQ ID NO: 222 - DNA, 29 bp, Homo sapiens
  source 1..29: mol_type = genomic DNA
gagaaagcgctgcaggaataccgcaaaaa

SEQ ID NO: 223 - DNA, 22 bp, Homo sapiens
  source 1..22: mol_type = genomic DNA
accttcggccatggggcaaata

SEQ ID NO: 224 - DNA, 27 bp, Homo sapiens
  source 1..27: mol_type = genomic DNA
aacgttcaccttgtctaccatcaagac

SEQ ID NO: 225 - DNA, 27 bp, Homo sapiens
  source 1..27: mol_type = genomic DNA
cggaaaacttcgaggaattgctcaaag

SEQ ID NO: 226 - DNA, 30 bp, Homo sapiens
  source 1..30: mol_type = genomic DNA
atttatatttggcatactttgtgcatgcag

SEQ ID NO: 227 - DNA, 26 bp, Homo sapiens
  source 1..26: mol_type = genomic DNA
ggctgcttccatcttttccagcaaat

SEQ ID NO: 228 - DNA, 22 bp, Homo sapiens
  source 1..22: mol_type = genomic DNA
actcacggctgcttggagcgtc

SEQ ID NO: 229 - DNA, 27 bp, Homo sapiens
  source 1..27: mol_type = genomic DNA
ctgcggtacgtgctcccgcctccgact

SEQ ID NO: 230 - DNA, 22 bp, Homo sapiens
  source 1..22: mol_type = genomic DNA
acgaggtcacctccatcctgcg

SEQ ID NO: 231 - DNA, 26 bp, Homo sapiens
  source 1..26: mol_type = genomic DNA
cctgcttcttacatattccaccccga

SEQ ID NO: 232 - DNA, 22 bp, Homo sapiens
  source 1..22: mol_type = genomic DNA
gcatcagaggcccccttagggc

SEQ ID NO: 233 - DNA, 26 bp, Homo sapiens
  source 1..26: mol_type = genomic DNA
ctgctggtcagcagcctctctccagt

SEQ ID NO: 234 - DNA, 27 bp, Homo sapiens
  source 1..27: mol_type = genomic DNA
cttatgggattgacagagaaactgatt

SEQ ID NO: 235 - DNA, 28 bp, Homo sapiens
  source 1..28: mol_type = genomic DNA
gacccctatgcgagaacatatctttaag

SEQ ID NO: 236 - DNA, 26 bp, Homo sapiens
  source 1..26: mol_type = genomic DNA
tgcctttgttgggaaatgttttgtcc

SEQ ID NO: 237 - DNA, 27 bp, Homo sapiens
  source 1..27: mol_type = genomic DNA
gcacgccgaccggcgccgggagatcct

SEQ ID NO: 238 - DNA, 30 bp, Homo sapiens
  source 1..30: mol_type = genomic DNA
cgccacaccgtcttctggaacagttcaaat

SEQ ID NO: 239 - DNA, 28 bp, Homo sapiens
  source 1..28: mol_type = genomic DNA
acctgcacaacgccgagttgagcaagat

SEQ ID NO: 240 - DNA, 24 bp, Homo sapiens
  source 1..24: mol_type = genomic DNA
cacccagcatcaaggggctgtcaa

SEQ ID NO: 241 - DNA, 25 bp, Homo sapiens
  source 1..25: mol_type = genomic DNA
gcgggaataagtaccagaccattga

SEQ ID NO: 242 - DNA, 22 bp, Homo sapiens
  source 1..22: mol_type = genomic DNA
ggcccactgccgtgtacttcct

SEQ ID NO: 243 - DNA, 27 bp, Homo sapiens
  source 1..27: mol_type = genomic DNA
ctaccatggaggagtaccatcgccact

SEQ ID NO: 244 - DNA, 22 bp, Homo sapiens
  source 1..22: mol_type = genomic DNA
ctgtcccgcctggcgtcccttc

SEQ ID NO: 245 - DNA, 25 bp, Homo sapiens
  source 1..25: mol_type = genomic DNA
aagtgaagctaaaactctacgcgct

SEQ ID NO: 246 - DNA, 26 bp, Homo sapiens
  source 1..26: mol_type = genomic DNA
tgccacctggacatcatttggatcaa

SEQ ID NO: 247 - DNA, 26 bp, Homo sapiens
  source 1..26: mol_type = genomic DNA
atacggagcactttcaaatatgccag

SEQ ID NO: 248 - DNA, 30 bp, Homo sapiens
  source 1..30: mol_type = genomic DNA
ccttctgaaaaatcttttcaagatattctg

SEQ ID NO: 249 - DNA, 29 bp, Homo sapiens
  source 1..29: mol_type = genomic DNA
aaccaaaagttgatagaaactggagaaag

SEQ ID NO: 250 - DNA, 29 bp, Homo sapiens
  source 1..29: mol_type = genomic DNA
tgctgcccgccggctgccgggcgctggaa

SEQ ID NO: 251 - DNA, 27 bp, Homo sapiens
  source 1..27: mol_type = genomic DNA
acttttgtgatggattcctaagtggaa

SEQ ID NO: 252 - DNA, 23 bp, Homo sapiens
  source 1..23: mol_type = genomic DNA
gcaaactgttgcctgctaagcgt

SEQ ID NO: 253 - DNA, 27 bp, Homo sapiens
  source 1..27: mol_type = genomic DNA
ggagggctccctggctttatctgtaca

SEQ ID NO: 254 - DNA, 26 bp, Homo sapiens
  source 1..26: mol_type = genomic DNA
aaagacctgtggcaaaagaggcagaa

SEQ ID NO: 255 - DNA, 22 bp, Homo sapiens
  source 1..22: mol_type = genomic DNA
cacgccgagtcctactccagcg

SEQ ID NO: 256 - DNA, 27 bp, Homo sapiens
  source 1..27: mol_type = genomic DNA
cctgattcaagactcctctgctttgga

SEQ ID NO: 257 - DNA, 23 bp, Homo sapiens
  source 1..23: mol_type = genomic DNA
ataagggtgacagcaacagctcg

SEQ ID NO: 258 - DNA, 28 bp, Homo sapiens
  source 1..28: mol_type = genomic DNA
gcagcctgcccttccccttcaacctctt

SEQ ID NO: 259 - DNA, 25 bp, Homo sapiens
  source 1..25: mol_type = genomic DNA
gatccggaagaaatatccggacagg

SEQ ID NO: 260 - DNA, 27 bp, Homo sapiens
  source 1..27: mol_type = genomic DNA
agtttgggattgagttttgctgctgtg

SEQ ID NO: 261 - DNA, 26 bp, Homo sapiens
  source 1..26: mol_type = genomic DNA
aggtgaaaccaacagccagtgatatg

SEQ ID NO: 262 - DNA, 29 bp, Homo sapiens
  source 1..29: mol_type = genomic DNA
tatactccaaatatgcaaatggaattgaa

SEQ ID NO: 263 - DNA, 26 bp, Homo sapiens
  source 1..26: mol_type = genomic DNA
ctgcttggcgccctgctctgcgcaca

SEQ ID NO: 264 - DNA, 28 bp, Homo sapiens
  source 1..28: mol_type = genomic DNA
tcgtctcgcagagccggggacaagagaa

SEQ ID NO: 265 - DNA, 29 bp, Homo sapiens
  source 1..29: mol_type = genomic DNA
tgatgaggaattcatagaaagcaataaaa

SEQ ID NO: 266 - DNA, 28 bp, Homo sapiens
  source 1..28: mol_type = genomic DNA
gaaatctgcagtatgacctccactactg

SEQ ID NO: 267 - DNA, 24 bp, Homo sapiens
  source 1..24: mol_type = genomic DNA
ggggacgccgcgacgggaacttga

SEQ ID NO: 268 - DNA, 28 bp, Homo sapiens
  source 1..28: mol_type = genomic DNA
cctttcaaaatgaagcccataggacttc

SEQ ID NO: 269 - DNA, 27 bp, Homo sapiens
  source 1..27: mol_type = genomic DNA
ttcaccgacatagtcattatgccgaag

SEQ ID NO: 270 - DNA, 23 bp, Homo sapiens
  source 1..23: mol_type = genomic DNA
tcctgcattgctgccctggctat

SEQ ID NO: 271 - DNA, 27 bp, Homo sapiens
  source 1..27: mol_type = genomic DNA
gtccaaatcaggatccactgcaaggaa

SEQ ID NO: 272 - DNA, 28 bp, Homo sapiens
  source 1..28: mol_type = genomic DNA
gtgaaggcggcatcattatcaatatgtc

SEQ ID NO: 273 - DNA, 25 bp, Homo sapiens
  source 1..25: mol_type = genomic DNA
ggacacgctgcaatctagtgacaaa

SEQ ID NO: 274 - DNA, 26 bp, Homo sapiens
  source 1..26: mol_type = genomic DNA
aatccaaagatggtcaaggtcgcaag

SEQ ID NO: 275 - DNA, 23 bp, Homo sapiens
  source 1..23: mol_type = genomic DNA
cgcgatcgggcttagtcggagct

SEQ ID NO: 276 - DNA, 24 bp, Homo sapiens
  source 1..24: mol_type = genomic DNA
aactcttcgccagcatatcatccc

SEQ ID NO: 277 - DNA, 29 bp, Homo sapiens
  source 1..29: mol_type = genomic DNA
atatgtaaaagaagcagaaaaccttaaga

SEQ ID NO: 278 - DNA, 24 bp, Homo sapiens
  source 1..24: mol_type = genomic DNA
cagcagggaggtgggcggcagcgt

SEQ ID NO: 279 - DNA, 28 bp, Homo sapiens
  source 1..28: mol_type = genomic DNA
tcatcctagcaaacaacagtttgtcttc

SEQ ID NO: 280 - DNA, 25 bp, Homo sapiens
  source 1..25: mol_type = genomic DNA
tgtgataggagccccgttctcacaa

SEQ ID NO: 281 - DNA, 27 bp, Homo sapiens
  source 1..27: mol_type = genomic DNA
ttcggctacgccgtggacttccacata

SEQ ID NO: 282 - DNA, 27 bp, Homo sapiens
  source 1..27: mol_type = genomic DNA
gaaatagctcatgggaacccagaagag

SEQ ID NO: 283 - DNA, 27 bp, Homo sapiens
  source 1..27: mol_type = genomic DNA
cattgacatactcatgacacatggacc

SEQ ID NO: 284 - DNA, 26 bp, Homo sapiens
  source 1..26: mol_type = genomic DNA
atgtccccatgctcctgcgccagcaa

SEQ ID NO: 285 - DNA, 30 bp, Homo sapiens
  source 1..30: mol_type = genomic DNA
gaatttccagattgatgtatatgaagctag

SEQ ID NO: 286 - DNA, 26 bp, Homo sapiens
  source 1..26: mol_type = genomic DNA
cacaagaccgacctcaaccccgacaa

SEQ ID NO: 287 - DNA, 29 bp, Homo sapiens
  source 1..29: mol_type = genomic DNA
attacctaaaggacccatcacttcttctg

SEQ ID NO: 288 - DNA, 27 bp, Homo sapiens
  source 1..27: mol_type = genomic DNA
cttctcctttgggatcgttctctgtga

SEQ ID NO: 289 - DNA, 25 bp, Homo sapiens
  source 1..25: mol_type = genomic DNA
aaaggtggctaaggacctcaaccca

SEQ ID NO: 290 - DNA, 26 bp, Homo sapiens
  source 1..26: mol_type = genomic DNA
gtttcccatacaaacactggactgca

SEQ ID NO: 291 - DNA, 27 bp, Homo sapiens
  source 1..27: mol_type = genomic DNA
cgacgtctggagcctgggcatcaccat

SEQ ID NO: 292 - DNA, 27 bp, Homo sapiens
  source 1..27: mol_type = genomic DNA
ggggagggctacatcgacttccgcatt

SEQ ID NO: 293 - DNA, 27 bp, Homo sapiens
  source 1..27: mol_type = genomic DNA
gggcaactcgctggtcatgttcgtgat

SEQ ID NO: 294 - DNA, 27 bp, Homo sapiens
  source 1..27: mol_type = genomic DNA
ctggagcccacagagcctgggcctctt

SEQ ID NO: 295 - DNA, 22 bp, Homo sapiens
  source 1..22: mol_type = genomic DNA
cagaaacctgggcaagacacct

SEQ ID NO: 296 - DNA, 27 bp, Homo sapiens
  source 1..27: mol_type = genomic DNA
ttgtctgtaaggaacacgaagctatga

SEQ ID NO: 297 - DNA, 23 bp, Homo sapiens
  source 1..23: mol_type = genomic DNA
ggaaggagattgacccaccgttc

SEQ ID NO: 298 - DNA, 22 bp, Homo sapiens
  source 1..22: mol_type = genomic DNA
tgttcgcgatcctgccggagcc

SEQ ID NO: 299 - DNA, 22 bp, Homo sapiens
  source 1..22: mol_type = genomic DNA
gggcgcgcgagttcagccgcct

SEQ ID NO: 300 - DNA, 26 bp, Homo sapiens
  source 1..26: mol_type = genomic DNA
tatttcagttcctgccaagacctcct

SEQ ID NO: 301 - DNA, 22 bp, Homo sapiens
  source 1..22: mol_type = genomic DNA
gggaggggaccatcggggtcgg

SEQ ID NO: 302 - DNA, 28 bp, Homo sapiens
  source 1..28: mol_type = genomic DNA
gcagggtaaccacgaccagcttaaagaa

SEQ ID NO: 303 - DNA, 30 bp, Homo sapiens
  source 1..30: mol_type = genomic DNA
tagtaatatgggtacaggtacatttggacc

SEQ ID NO: 304 - DNA, 26 bp, Homo sapiens
  source 1..26: mol_type = genomic DNA
cgcagcttaggcagcggaggttctgt

SEQ ID NO: 305 - DNA, 26 bp, Homo sapiens
  source 1..26: mol_type = genomic DNA
cccgaggacaacctggagatcgttct

SEQ ID NO: 306 - DNA, 26 bp, Homo sapiens
  source 1..26: mol_type = genomic DNA
tgagggtccacaccgcgagggaagat

SEQ ID NO: 307 - DNA, 28 bp, Homo sapiens
  source 1..28: mol_type = genomic DNA
ggttctagaaatgtctcttgaagtttgc

SEQ ID NO: 308 - DNA, 26 bp, Homo sapiens
  source 1..26: mol_type = genomic DNA
gagagcacagtgtcaggcaacggaat

SEQ ID NO: 309 - DNA, 26 bp, Homo sapiens
  source 1..26: mol_type = genomic DNA
catcgagaaggcgtctgcgagaccat

SEQ ID NO: 310 - DNA, 25 bp, Homo sapiens
  source 1..25: mol_type = genomic DNA
tagtcgtatcaggggtcgggaccaa

SEQ ID NO: 311 - DNA, 23 bp, Homo sapiens
  source 1..23: mol_type = genomic DNA
aggcgaggagtgccaccccggca

SEQ ID NO: 312 - DNA, 27 bp, Homo sapiens
  source 1..27: mol_type = genomic DNA
taatgcttatcctgacctaagaagctg

SEQ ID NO: 313 - DNA, 27 bp, Homo sapiens
  source 1..27: mol_type = genomic DNA
agggatcgaagctggaaatattaatat

SEQ ID NO: 314 - DNA, 23 bp, Homo sapiens
  source 1..23: mol_type = genomic DNA
gacccgcggttcctcatcctcct

SEQ ID NO: 315 - DNA, 25 bp, Homo sapiens
  source 1..25: mol_type = genomic DNA
cccctgctcggctacaaaaaccaaa

SEQ ID NO: 316 - DNA, 27 bp, Homo sapiens
  source 1..27: mol_type = genomic DNA
ggggcttctccttcgagaactgccaaa

SEQ ID NO: 317 - DNA, 25 bp, Homo sapiens
  source 1..25: mol_type = genomic DNA
tgcagcagtggattctcgggcctca

SEQ ID NO: 318 - DNA, 26 bp, Homo sapiens
  source 1..26: mol_type = genomic DNA
cttttgccctggccaagggcttcaca

SEQ ID NO: 319 - DNA, 25 bp, Homo sapiens
  source 1..25: mol_type = genomic DNA
gcgcggccgagtccccgtacggcca

SEQ ID NO: 320 - DNA, 30 bp, Homo sapiens
  source 1..30: mol_type = genomic DNA
cgccgggtggagattctcagtgaaggaaat

SEQ ID NO: 321 - DNA, 26 bp, Homo sapiens
  source 1..26: mol_type = genomic DNA
accagacctcctcttggcttcgagat

SEQ ID NO: 322 - DNA, 23 bp, Homo sapiens
  source 1..23: mol_type = genomic DNA
attgtaggtggtgtccagctcca

SEQ ID NO: 323 - DNA, 28 bp, Homo sapiens
  source 1..28: mol_type = genomic DNA
ctagcgttcctgctggccctgggacaaa

SEQ ID NO: 324 - DNA, 25 bp, Homo sapiens
  source 1..25: mol_type = genomic DNA
tgacccgggagctgcccagcttctt

SEQ ID NO: 325 - DNA, 27 bp, Homo sapiens
  source 1..27: mol_type = genomic DNA
tcctggaaatatggaagcactttgacg

SEQ ID NO: 326 - DNA, 28 bp, Homo sapiens
  source 1..28: mol_type = genomic DNA
cccgtttgccgacccggatctcaacaat

SEQ ID NO: 327 - DNA, 26 bp, Homo sapiens
  source 1..26: mol_type = genomic DNA
cggatgaaactctgagcaatgttgag

SEQ ID NO: 328 - DNA, 24 bp, Homo sapiens
  source 1..24: mol_type = genomic DNA
ggccgtgaaggccctgaaggccct

SEQ ID NO: 329 - DNA, 25 bp, Homo sapiens
  source 1..25: mol_type = genomic DNA
tttcacccaccactcagcagctgta

SEQ ID NO: 330 - DNA, 22 bp, Homo sapiens
  source 1..22: mol_type = genomic DNA
cgcctgaagccatcgtcacgga

SEQ ID NO: 331 - DNA, 29 bp, Homo sapiens
  source 1..29: mol_type = genomic DNA
gagttttgcgaaagattttcctactatgg

SEQ ID NO: 332 - DNA, 29 bp, Homo sapiens
  source 1..29: mol_type = genomic DNA
ataatctcaatctgtgtgtttgtcttaac

SEQ ID NO: 333 - DNA, 28 bp, Homo sapiens
  source 1..28: mol_type = genomic DNA
gaggcagccccagaatcagcaaaaagta

SEQ ID NO: 334 - DNA, 25 bp, Homo sapiens
  source 1..25: mol_type = genomic DNA
acggcctgcaagctgctcaacatca

SEQ ID NO: 335 - DNA, 28 bp, Homo sapiens
  source 1..28: mol_type = genomic DNA
caccttgggctgtggaaggctctggaaa

SEQ ID NO: 336 - DNA, 30 bp, Homo sapiens
  source 1..30: mol_type = genomic DNA
ggatcagcgtcgccagggtctggaagattt

SEQ ID NO: 337 - DNA, 22 bp, Homo sapiens
  source 1..22: mol_type = genomic DNA
gtccactggtctggccacaaca

SEQ ID NO: 338 - DNA, 27 bp, Homo sapiens
  source 1..27: mol_type = genomic DNA
aaatctaagaagtttcgcagacctgac

SEQ ID NO: 339 - DNA, 22 bp, Homo sapiens
  source 1..22: mol_type = genomic DNA
aataaggagcagctcgaggcca

SEQ ID NO: 340 - DNA, 26 bp, Homo sapiens
  source 1..26: mol_type = genomic DNA
aaacttacgtggctactcagcatcga

SEQ ID NO: 341 - DNA, 26 bp, Homo sapiens
  source 1..26: mol_type = genomic DNA
gaaatcccgagtggcggctcaaaact

SEQ ID NO: 342 - DNA, 22 bp, Homo sapiens
  source 1..22: mol_type = genomic DNA
tccaccatcccgggaccccggc

SEQ ID NO: 343 - DNA, 27 bp, Homo sapiens
  source 1..27: mol_type = genomic DNA
ggaggcgctcatggccgaccacaggaa

SEQ ID NO: 344 - DNA, 28 bp, Homo sapiens
  source 1..28: mol_type = genomic DNA
actctctgcttacttttgtctgagatgg

SEQ ID NO: 345 - DNA, 27 bp, Homo sapiens
  source 1..27: mol_type = genomic DNA
gcagtcaactggagagagttccgattt

SEQ ID NO: 346 - DNA, 26 bp, Homo sapiens
  source 1..26: mol_type = genomic DNA
gaaggtgggtctgaatctagcaccat

SEQ ID NO: 347 - DNA, 23 bp, Homo sapiens
  source 1..23: mol_type = genomic DNA
acctgttccccctgcgtccagca

SEQ ID NO: 348 - DNA, 26 bp, Homo sapiens
  source 1..26: mol_type = genomic DNA
ctgtcctccagctctgctgaggagta

SEQ ID NO: 349 - DNA, 27 bp, Homo sapiens
  source 1..27: mol_type = genomic DNA
tgagagcttcagtgacgccaaggacaa

SEQ ID NO: 350 - DNA, 25 bp, Homo sapiens
  source 1..25: mol_type = genomic DNA
gcttcttcagtttcccagaactgca

SEQ ID NO: 351 - DNA, 27 bp, Homo sapiens
  source 1..27: mol_type = genomic DNA
cttgcctggagatagcctttgcgatat

SEQ ID NO: 352 - DNA, 26 bp, Homo sapiens
  source 1..26: mol_type = genomic DNA
ccggatgaaaccagctctgtccctgt

SEQ ID NO: 353 - DNA, 26 bp, Homo sapiens
  source 1..26: mol_type = genomic DNA
aatggctggtggagaggagaagtaaa

SEQ ID NO: 354 - DNA, 26 bp, Homo sapiens
  source 1..26: mol_type = genomic DNA
cggggcgcgctctcgcctctcctgca

SEQ ID NO: 355 - DNA, 28 bp, Homo sapiens
  source 1..28: mol_type = genomic DNA
gacagtgtcgtcgtagaaagagaacgta

SEQ ID NO: 356 - DNA, 27 bp, Homo sapiens
  source 1..27: mol_type = genomic DNA
gacaaattggttttctttgtgaatggc

SEQ ID NO: 357 - DNA, 23 bp, Homo sapiens
  source 1..23: mol_type = genomic DNA
ctgtctgtgcacacagaaaaccc

SEQ ID NO: 358 - DNA, 29 bp, Homo sapiens
  source 1..29: mol_type = genomic DNA
gtgattcgtcaacccgtgggcaggatttt

SEQ ID NO: 359 - DNA, 23 bp, Homo sapiens
  source 1..23: mol_type = genomic DNA
cactttacggagaacatggagga

SEQ ID NO: 360 - DNA, 24 bp, Homo sapiens
  source 1..24: mol_type = genomic DNA
acattcacggcatggtgtaactcc

SEQ ID NO: 361 - DNA, 26 bp, Homo sapiens
  source 1..26: mol_type = genomic DNA
atggcacgaatccaagagtgggaaaa

SEQ ID NO: 362 - DNA, 29 bp, Homo sapiens
  source 1..29: mol_type = genomic DNA
gcaactatgaagagaaaagctactaataa

SEQ ID NO: 363 - DNA, 27 bp, Homo sapiens
  source 1..27: mol_type = genomic DNA
cacaagggaatttgattcagattctct

SEQ ID NO: 364 - DNA, 23 bp, Homo sapiens
  source 1..23: mol_type = genomic DNA
tttgtgaaaatccatgccccctg

SEQ ID NO: 365 - DNA, 26 bp, Homo sapiens
  source 1..26: mol_type = genomic DNA
agcttcaagaagcagtcgtttgtgct

SEQ ID NO: 366 - DNA, 29 bp, Homo sapiens
  source 1..29: mol_type = genomic DNA
tcatcagagcaagaaaaagaacaagagac

SEQ ID NO: 367 - DNA, 29 bp, Homo sapiens
  source 1..29: mol_type = genomic DNA
attctacgtaatattttatggctgcctgg

SEQ ID NO: 368 - DNA, 23 bp, Homo sapiens
  source 1..23: mol_type = genomic DNA
gatcatcaccatgctggtcgcca

SEQ ID NO: 369 - DNA, 23 bp, Homo sapiens
  source 1..23: mol_type = genomic DNA
caagtgctcacaggcaaaagact

SEQ ID NO: 370 - DNA, 29 bp, Homo sapiens
  source 1..29: mol_type = genomic DNA
ggatttttccaagctacccaaaatactcg

SEQ ID NO: 371 - DNA, 22 bp, Homo sapiens
  source 1..22: mol_type = genomic DNA
gagaagcggtggagtgtgtcct

SEQ ID NO: 372 - DNA, 25 bp, Homo sapiens
  source 1..25: mol_type = genomic DNA
cgaatctacggacattttgctttca

SEQ ID NO: 373 - DNA, 26 bp, Homo sapiens
  source 1..26: mol_type = genomic DNA
gccaaagctgtttgatggatgctact

SEQ ID NO: 374 - DNA, 27 bp, Homo sapiens
  source 1..27: mol_type = genomic DNA
gcacctgaaggagcgcttggccaatga

SEQ ID NO: 375 - DNA, 25 bp, Homo sapiens
  source 1..25: mol_type = genomic DNA
cccaaggctcctgaccagtgaacaa

SEQ ID NO: 376 - DNA, 23 bp, Homo sapiens
  source 1..23: mol_type = genomic DNA
tcctgaacgccccacctgttcca

SEQ ID NO: 377 - DNA, 27 bp, Homo sapiens
  source 1..27: mol_type = genomic DNA
tgaccaactaaatgacagatgtgtgag

SEQ ID NO: 378 - DNA, 22 bp, Homo sapiens
  source 1..22: mol_type = genomic DNA
gctgacagctgtatccagttca

SEQ ID NO: 379 - DNA, 24 bp, Homo sapiens
  source 1..24: mol_type = genomic DNA
ccgcgtcgtcaatatcagcagcat

SEQ ID NO: 380 - DNA, 25 bp, Homo sapiens
  source 1..25: mol_type = genomic DNA
ccatccaccggaaggttgctgaaga

SEQ ID NO: 381 - DNA, 27 bp, Homo sapiens
  source 1..27: mol_type = genomic DNA
aaatgcttttgctgtgatggtggactc

SEQ ID NO: 382 - DNA, 30 bp, Homo sapiens
  source 1..30: mol_type = genomic DNA
gcatttgaatatgaaattcgattttacact

SEQ ID NO: 383 - DNA, 27 bp, Homo sapiens
  source 1..27: mol_type = genomic DNA
tgctctgtgagctgtcagtctaggtta

SEQ ID NO: 384 - DNA, 27 bp, Homo sapiens
  source 1..27: mol_type = genomic DNA
agttctaggcctccagttccagactat

SEQ ID NO: 385 - DNA, 27 bp, Homo sapiens
  source 1..27: mol_type = genomic DNA
ttcttgaagcacatccaacttatccaa

SEQ ID NO: 386 - DNA, 24 bp, Homo sapiens
  source 1..24: mol_type = genomic DNA
tcatgcagaacaaccacattgcct

SEQ ID NO: 387 - DNA, 28 bp, Homo sapiens
  source 1..28: mol_type = genomic DNA
gcaaattgaactctatctaatttgcatg

SEQ ID NO: 388 - DNA, 26 bp, Homo sapiens
  source 1..26: mol_type = genomic DNA
ccgtgtgcgcaccacctacggcttct

SEQ ID NO: 389 - DNA, 28 bp, Homo sapiens
  source 1..28: mol_type = genomic DNA
atgatccaatgccctttgacattaaagc

SEQ ID NO: 390 - DNA, 22 bp, Homo sapiens
  source 1..22: mol_type = genomic DNA
atgaagccacgctccaggccat

SEQ ID NO: 391 - DNA, 23 bp, Homo sapiens
  source 1..23: mol_type = genomic DNA
gtggccttcccccagatgtacct

SEQ ID NO: 392 - DNA, 28 bp, Homo sapiens
  source 1..28: mol_type = genomic DNA
aaccctggccttaaaattccaaaagaag

SEQ ID NO: 393 - DNA, 25 bp, Homo sapiens
  source 1..25: mol_type = genomic DNA
gaggcagctgaggccagagcacttt

SEQ ID NO: 394 - DNA, 25 bp, Homo sapiens
  source 1..25: mol_type = genomic DNA
tcgctgtgggcgctgtcatgatgtt

SEQ ID NO: 395 - DNA, 26 bp, Homo sapiens
  source 1..26: mol_type = genomic DNA
gatgtgcttatgcaggattccaggtt

SEQ ID NO: 396 - DNA, 27 bp, Homo sapiens
  source 1..27: mol_type = genomic DNA
ctgtggctccaaactgcttcaactcat

SEQ ID NO: 397 - DNA, 27 bp, Homo sapiens
  source 1..27: mol_type = genomic DNA
ttaactgttgccttattaacccctccc

SEQ ID NO: 398 - DNA, 26 bp, Homo sapiens
  source 1..26: mol_type = genomic DNA
catataactgctcaacctgtccccga

SEQ ID NO: 399 - DNA, 24 bp, Homo sapiens
  source 1..24: mol_type = genomic DNA
tacaccgtgctccggctaatgatt

SEQ ID NO: 400 - DNA, 23 bp, Homo sapiens
  source 1..23: mol_type = genomic DNA
ggatgttgcttttgcacctacgg

SEQ ID NO: 401 - DNA, 26 bp, Homo sapiens
  source 1..26: mol_type = genomic DNA
cttcacagcaggaaggactcaaattg

SEQ ID NO: 402 - DNA, 28 bp, Homo sapiens
  source 1..28: mol_type = genomic DNA
ggctgtgggtaatattgtgaagttcttg

SEQ ID NO: 403 - DNA, 27 bp, Homo sapiens
  source 1..27: mol_type = genomic DNA
aatgtgatgctgaggaagattgctgtg

SEQ ID NO: 404 - DNA, 25 bp, Homo sapiens
  source 1..25: mol_type = genomic DNA
caagtcaatctgaaagtcccagcca

SEQ ID NO: 405 - DNA, 27 bp, Homo sapiens
  source 1..27: mol_type = genomic DNA
gctttgttaaccacccaaacacaagtg

SEQ ID NO: 406 - DNA, 27 bp, Homo sapiens
  source 1..27: mol_type = genomic DNA
ggagtccatagtatgtctgcagaaagc

SEQ ID NO: 407 - DNA, 27 bp, Homo sapiens
  source 1..27: mol_type = genomic DNA
tgcctgtctggggaggtggaaacaagt

SEQ ID NO: 408 - DNA, 24 bp, Homo sapiens
  source 1..24: mol_type = genomic DNA
cattgtgaccaccacgagagtgaa

SEQ ID NO: 409 - DNA, 26 bp, Homo sapiens
  source 1..26: mol_type = genomic DNA
gtttgatgacatggcagacactgagt

SEQ ID NO: 410 - DNA, 27 bp, Homo sapiens
  source 1..27: mol_type = genomic DNA
cctaggtccccagccgctagagctgaa

SEQ ID NO: 411 - DNA, 28 bp, Homo sapiens
  source 1..28: mol_type = genomic DNA
ttctggaggtctattacacaagcttgag

SEQ ID NO: 412 - DNA, 27 bp, Homo sapiens
  source 1..27: mol_type = genomic DNA
cagtacattcccgccagaaggtgtttt

SEQ ID NO: 413 - DNA, 27 bp, Homo sapiens
  source 1..27: mol_type = genomic DNA
gtggccaggcatggaaggagcaaagaa

SEQ ID NO: 414 - DNA, 26 bp, Homo sapiens
  source 1..26: mol_type = genomic DNA
gtctctggaaatttgacacagagtgc

SEQ ID NO: 415 - DNA, 28 bp, Homo sapiens
  source 1..28: mol_type = genomic DNA
gataaagtccttgatgaaacctgatccc

SEQ ID NO: 416 - DNA, 25 bp, Homo sapiens
  source 1..25: mol_type = genomic DNA
accatacatgtgcagctgaatgact

SEQ ID NO: 417 - DNA, 22 bp, Homo sapiens
  source 1..22: mol_type = genomic DNA
cgctgacgctggcggagaagcg

SEQ ID NO: 418 - DNA, 27 bp, Homo sapiens
  source 1..27: mol_type = genomic DNA
ccctggcagtccaatgtcctggcaaca

SEQ ID NO: 419 - DNA, 27 bp, Homo sapiens
  source 1..27: mol_type = genomic DNA
cgtacccgtgcgcagaggacgaggagt

SEQ ID NO: 420 - DNA, 25 bp, Homo sapiens
  source 1..25: mol_type = genomic DNA
gggctgctgtcccgatctgtgctct

SEQ ID NO: 421 - DNA, 23 bp, Homo sapiens
  source 1..23: mol_type = genomic DNA
ggttggcttcaatgctgaggaag

SEQ ID NO: 422 - DNA, 27 bp, Homo sapiens
  source 1..27: mol_type = genomic DNA
tgctaactttgagtacatcatcgcaga

SEQ ID NO: 423 - DNA, 24 bp, Homo sapiens
  source 1..24: mol_type = genomic DNA
ccactgaaggaccttgtaacatgc

SEQ ID NO: 424 - DNA, 26 bp, Homo sapiens
  source 1..26: mol_type = genomic DNA
cagacggtgccctatggactgtccaa

SEQ ID NO: 425 - DNA, 27 bp, Homo sapiens
  source 1..27: mol_type = genomic DNA
tgataaatggactcgaacaacttttga

SEQ ID NO: 426 - DNA, 22 bp, Homo sapiens
  source 1..22: mol_type = genomic DNA
tgattgacatcggctctggccc

SEQ ID NO: 427 - DNA, 29 bp, Homo sapiens
  source 1..29: mol_type = genomic DNA
gagttgctgagagctaaattaattgaatg

SEQ ID NO: 428 - DNA, 26 bp, Homo sapiens
  source 1..26: mol_type = genomic DNA
agaccctcatggacacaaaatgggta

SEQ ID NO: 429 - DNA, 26 bp, Homo sapiens
  source 1..26: mol_type = genomic DNA
tcagaaggaaagactccaaaggtgga

SEQ ID NO: 430 - DNA, 23 bp, Homo sapiens
  source 1..23: mol_type = genomic DNA
ctaaaaggaagaagcccctgccc

SEQ ID NO: 431 - DNA, 24 bp, Homo sapiens
  source 1..24: mol_type = genomic DNA
gctggatacttcaccaaagcgtct

SEQ ID NO: 432 - DNA, 27 bp, Homo sapiens
  source 1..27: mol_type = genomic DNA
agtcaatgagtactcctcagaactgga

SEQ ID NO: 433 - DNA, 24 bp, Homo sapiens
  source 1..24: mol_type = genomic DNA
aattccgggtagatatgcctggct

SEQ ID NO: 434 - DNA, 27 bp, Homo sapiens
  source 1..27: mol_type = genomic DNA
ggagtttgtgaccaagaacttcaagag

SEQ ID NO: 435 - DNA, 27 bp, Homo sapiens
  source 1..27: mol_type = genomic DNA
tcaattcgtcataatctgtccctacac

SEQ ID NO: 436 - DNA, 25 bp, Homo sapiens
  source 1..25: mol_type = genomic DNA
aactgcagcagctctggaaagaagt

SEQ ID NO: 437 - DNA, 26 bp, Homo sapiens
  source 1..26: mol_type = genomic DNA
gctccaaaagccagggtgcctgatct

SEQ ID NO: 438 - DNA, 28 bp, Homo sapiens
  source 1..28: mol_type = genomic DNA
ctgcattgtcatgacatttccaacactg

SEQ ID NO: 439 - DNA, 26 bp, Homo sapiens
  source 1..26: mol_type = genomic DNA
cttgggacccagcactagcccaaatt

SEQ ID NO: 440 - DNA, 29 bp, Homo sapiens
  source 1..29: mol_type = genomic DNA
aaaagcatatgaaagaattcaaggttttg

SEQ ID NO: 441 - DNA, 25 bp, Homo sapiens
  source 1..25: mol_type = genomic DNA
ggccagcagccccgagtgtgcttgt

SEQ ID NO: 442 - DNA, 23 bp, Homo sapiens
  source 1..23: mol_type = genomic DNA
agtggcaccatttacgagtacgg

SEQ ID NO: 443 - DNA, 26 bp, Homo sapiens
  source 1..26: mol_type = genomic DNA
tgtttggaaacctacaaggcctcaca

SEQ ID NO: 444 - DNA, 23 bp, Homo sapiens
  source 1..23: mol_type = genomic DNA
caatgagtgcagccaggatgaga

SEQ ID NO: 445 - DNA, 23 bp, Homo sapiens
  source 1..23: mol_type = genomic DNA
gaaggcccaaaatgaccctctta

SEQ ID NO: 446 - DNA, 27 bp, Homo sapiens
  source 1..27: mol_type = genomic DNA
agagggtccaacgtatctcttacattg

SEQ ID NO: 447 - DNA, 26 bp, Homo sapiens
  source 1..26: mol_type = genomic DNA
tacagagggcaaagatggatccaaag

SEQ ID NO: 448 - DNA, 24 bp, Homo sapiens
  source 1..24: mol_type = genomic DNA
cgggctcaaggaacccaagagagt

SEQ ID NO: 449 - DNA, 25 bp, Homo sapiens
  source 1..25: mol_type = genomic DNA
ccttattccactgctggggattgat

SEQ ID NO: 450 - DNA, 25 bp, Homo sapiens
  source 1..25: mol_type = genomic DNA
gcagccggtttattgtgcttcaaag

SEQ ID NO: 451 - DNA, 29 bp, Homo sapiens
  source 1..29: mol_type = genomic DNA
tttctcatgaagaactagacgactcttgg

SEQ ID NO: 452 - DNA, 26 bp, Homo sapiens
  source 1..26: mol_type = genomic DNA
aaaaggaccccacgaagtgttggata

SEQ ID NO: 453 - DNA, 30 bp, Homo sapiens
  source 1..30: mol_type = genomic DNA
gtgactaggacacccgggtgggctactttt

SEQ ID NO: 454 - DNA, 27 bp, Homo sapiens
  source 1..27: mol_type = genomic DNA
cagttgagtctgcaagactgggaggaa

SEQ ID NO: 455 - DNA, 27 bp, Homo sapiens
  source 1..27: mol_type = genomic DNA
ttcagatgtagcggataatggaactct

SEQ ID NO: 456 - DNA, 24 bp, Homo sapiens
  source 1..24: mol_type = genomic DNA
aatcccaatggggaagtcgatgct

SEQ ID NO: 457 - DNA, 26 bp, Homo sapiens
  source 1..26: mol_type = genomic DNA
ggatgcaaagaatgtgaggaactgga

SEQ ID NO: 458 - DNA, 27 bp, Homo sapiens
  source 1..27: mol_type = genomic DNA
gagcatggtcccgctgccataagagaa

SEQ ID NO: 459 - DNA, 23 bp, Homo sapiens
  source 1..23: mol_type = genomic DNA
gggggcgcccaaagccaacacca

SEQ ID NO: 460 - DNA, 25 bp, Homo sapiens
  source 1..25: mol_type = genomic DNA
tggtcttcgaggccctgcacaatct

SEQ ID NO: 461 - DNA, 25 bp, Homo sapiens
  source 1..25: mol_type = genomic DNA
ttttcgagactgggttccaaaggag

SEQ ID NO: 462 - DNA, 26 bp, Homo sapiens
  source 1..26: mol_type = genomic DNA
atgttctctggatgtcagctgagtca

SEQ ID NO: 463 - DNA, 23 bp, Homo sapiens
  source 1..23: mol_type = genomic DNA
cacacgtggaagaagcattaact

SEQ ID NO: 464 - DNA, 23 bp, Homo sapiens
  source 1..23: mol_type = genomic DNA
cctggaccccaactacgtgctga

SEQ ID NO: 465 - DNA, 24 bp, Homo sapiens
  source 1..24: mol_type = genomic DNA
aatcacaaatgacggcccagaaca

SEQ ID NO: 466 - DNA, 27 bp, Homo sapiens
  source 1..27: mol_type = genomic DNA
cattgggcaggtgtatgcagatcctga

SEQ ID NO: 467 - DNA, 24 bp, Homo sapiens
  source 1..24: mol_type = genomic DNA
ccagctgcagtcagcaagaggtgt

SEQ ID NO: 468 - DNA, 26 bp, Homo sapiens
  source 1..26: mol_type = genomic DNA
gtgccaaacaacatccctccagatat

SEQ ID NO: 469 - DNA, 23 bp, Homo sapiens
  source 1..23: mol_type = genomic DNA
atggccatcctgcggttccctta

SEQ ID NO: 470 - DNA, 24 bp, Homo sapiens
  source 1..24: mol_type = genomic DNA
cggagaggacgacgagacggagga

SEQ ID NO: 471 - DNA, 27 bp, Homo sapiens
  source 1..27: mol_type = genomic DNA
caaagatgaagacagcaaccaacattt

SEQ ID NO: 472 - DNA, 22 bp, Homo sapiens
  source 1..22: mol_type = genomic DNA
gtgaggaacagtacccgtgcac

SEQ ID NO: 473 - DNA, 29 bp, Homo sapiens
  source 1..29: mol_type = genomic DNA
gactctggaggccccctgacctgtgagaa

SEQ ID NO: 474 - DNA, 22 bp, Homo sapiens
  source 1..22: mol_type = genomic DNA
gagctttgccgtcagatggctg

SEQ ID NO: 475 - DNA, 27 bp, Homo sapiens
  source 1..27: mol_type = genomic DNA
aatcaccatttgactgcagcaatttcg

SEQ ID NO: 476 - DNA, 27 bp, Homo sapiens
  source 1..27: mol_type = genomic DNA
attctgaaaccttccttgtatccctcc

SEQ ID NO: 477 - DNA, 26 bp, Homo sapiens
  source 1..26: mol_type = genomic DNA
aactgtctatcttgaccatgcaggtg

SEQ ID NO: 478 - DNA, 27 bp, Homo sapiens
  source 1..27: mol_type = genomic DNA
tagtgaccaccataaagatgtcaagcc

SEQ ID NO: 479 - DNA, 29 bp, Homo sapiens
  source 1..29: mol_type = genomic DNA
ttccaagacgggtgccaagtgatgagtat

SEQ ID NO: 480 - DNA, 22 bp, Homo sapiens
  source 1..22: mol_type = genomic DNA
cggtgctggctactgaccccct

SEQ ID NO: 481 - DNA, 25 bp, Homo sapiens
  source 1..25: mol_type = genomic DNA
ccctgaatcaagggaacaccagttt

SEQ ID NO: 482 - DNA, 26 bp, Homo sapiens
  source 1..26: mol_type = genomic DNA
cggctccgtggatgaccgtgggacct

SEQ ID NO: 483 - DNA, 26 bp, Homo sapiens
  source 1..26: mol_type = genomic DNA
tgtgttgagaagaaggtccttggaga

SEQ ID NO: 484 - DNA, 24 bp, Homo sapiens
  source 1..24: mol_type = genomic DNA
gagcctaagcctggagacctgatt

SEQ ID NO: 485 - DNA, 27 bp, Homo sapiens
  source 1..27: mol_type = genomic DNA
gatttagtatggctctgtgtgatcagg

SEQ ID NO: 486 - DNA, 22 bp, Homo sapiens
  source 1..22: mol_type = genomic DNA
cgcaggtctacgccccgcctcg

SEQ ID NO: 487 - DNA, 29 bp, Homo sapiens
  source 1..29: mol_type = genomic DNA
tacacctatgaagattataagaacactgc

SEQ ID NO: 488 - DNA, 23 bp, Homo sapiens
  source 1..23: mol_type = genomic DNA
acagattttgggcaccaaaaaga

SEQ ID NO: 489 - DNA, 25 bp, Homo sapiens
  source 1..25: mol_type = genomic DNA
aaacgcaagcaccacacctgtcctt

SEQ ID NO: 490 - DNA, 25 bp, Homo sapiens
  source 1..25: mol_type = genomic DNA
cattccagaccagtgtagtcctctg

SEQ ID NO: 491 - DNA, 25 bp, Homo sapiens
  source 1..25: mol_type = genomic DNA
ttgaagagcatatcagcgagcgaca

SEQ ID NO: 492 - DNA, 24 bp, Homo sapiens
  source 1..24: mol_type = genomic DNA
ccaaagcttcgtaccttggccaga

SEQ ID NO: 493 - DNA, 22 bp, Homo sapiens
  source 1..22: mol_type = genomic DNA
tgaccacaccccggtagccact

SEQ ID NO: 494 - DNA, 22 bp, Homo sapiens
  source 1..22: mol_type = genomic DNA
atcattggaacgcgtcctcccg

SEQ ID NO: 495 - DNA, 25 bp, Homo sapiens
  source 1..25: mol_type = genomic DNA
ggtgattgagattaacccttacctg

SEQ ID NO: 496 - DNA, 24 bp, Homo sapiens
  source 1..24: mol_type = genomic DNA
gcccacaagataatggctagctcc

SEQ ID NO: 497 - DNA, 24 bp, Homo sapiens
  source 1..24: mol_type = genomic DNA
ctacaagacgaccaccatcctgct

SEQ ID NO: 498 - DNA, 27 bp, Homo sapiens
  source 1..27: mol_type = genomic DNA
atccagttggcgaaggactttgaggat

SEQ ID NO: 499 - DNA, 28 bp, Homo sapiens
  source 1..28: mol_type = genomic DNA
ccaagagcccaaacctggagacctgatt

SEQ ID NO: 500 - DNA, 23 bp, Homo sapiens
  source 1..23: mol_type = genomic DNA
atgtgccagctgtccaaaattaa

SEQ ID NO: 501 - DNA, 27 bp, Homo sapiens
  source 1..27: mol_type = genomic DNA
cagaatagaactcgtagctcgtgactg

SEQ ID NO: 502 - DNA, 26 bp, Homo sapiens
  source 1..26: mol_type = genomic DNA
gatgaagctgctttccagaagctgat

SEQ ID NO: 503 - DNA, 30 bp, Homo sapiens
  source 1..30: mol_type = genomic DNA
attgaaggtaaagagctagaaaactttttc

SEQ ID NO: 504 - DNA, 28 bp, Homo sapiens
  source 1..28: mol_type = genomic DNA
cagttacacaagtgacaagaaatgttcc

SEQ ID NO: 505 - DNA, 29 bp, Homo sapiens
  source 1..29: mol_type = genomic DNA
aattaatatatgacagcagtctttgtgat

SEQ ID NO: 506 - DNA, 23 bp, Homo sapiens
  source 1..23: mol_type = genomic DNA
ctgacagtgtttggctgagccga

SEQ ID NO: 507 - DNA, 26 bp, Homo sapiens
  source 1..26: mol_type = genomic DNA
caatttttgaggaacgagcccacatc

SEQ ID NO: 508 - DNA, 26 bp, Homo sapiens
  source 1..26: mol_type = genomic DNA
acatcacaccagacatgatggtacag

SEQ ID NO: 509 - DNA, 28 bp, Homo sapiens
  source 1..28: mol_type = genomic DNA
ctgtacttcacaaatttcatcagctggg

SEQ ID NO: 510 - DNA, 24 bp, Homo sapiens
  source 1..24: mol_type = genomic DNA
cgccacagtcctgagcaatcgttt

SEQ ID NO: 511 - DNA, 26 bp, Homo sapiens
  source 1..26: mol_type = genomic DNA
catttttgccagcgttcagcatcttg

SEQ ID NO: 512 - DNA, 22 bp, Homo sapiens
  source 1..22: mol_type = genomic DNA
gccccagcaatgtgcagaagtg

SEQ ID NO: 513 - DNA, 28 bp, Homo sapiens
  source 1..28: mol_type = genomic DNA
ccttcaaagctggagtctgtcctcctaa

SEQ ID NO: 514 - DNA, 26 bp, Homo sapiens
  source 1..26: mol_type = genomic DNA
acttttgctttcagatagcagccttc

SEQ ID NO: 515 - DNA, 25 bp, Homo sapiens
  source 1..25: mol_type = genomic DNA
agctctatgactataacctggggag

SEQ ID NO: 516 - DNA, 26 bp, Homo sapiens
  source 1..26: mol_type = genomic DNA
cgaggacatcacctcacacatggaaa

SEQ ID NO: 517 - DNA, 29 bp, Homo sapiens
  source 1..29: mol_type = genomic DNA
ccaatatttcagaaacaagcttaatagga

SEQ ID NO: 518 - DNA, 25 bp, Homo sapiens
  source 1..25: mol_type = genomic DNA
ggtggctgcccaagagcatcatcaa

SEQ ID NO: 519 - DNA, 23 bp, Homo sapiens
  source 1..23: mol_type = genomic DNA
gcctcaacagtgctctacaggtc

SEQ ID NO: 520 - DNA, 27 bp, Homo sapiens
  source 1..27: mol_type = genomic DNA
tcctgagatcttcaccttcgaccctct

SEQ ID NO: 521 - DNA, 23 bp, Homo sapiens
  source 1..23: mol_type = genomic DNA
caaggagagcgccctggcgccct

SEQ ID NO: 522 - DNA, 27 bp, Homo sapiens
  source 1..27: mol_type = genomic DNA
aggtaagctctggtacctgcaagagtt

SEQ ID NO: 523 - DNA, 24 bp, Homo sapiens
  source 1..24: mol_type = genomic DNA
gaccctgatcttgtgtacagccca

SEQ ID NO: 524 - DNA, 26 bp, Homo sapiens
  source 1..26: mol_type = genomic DNA
tagagacagccatgggcatgatcata

SEQ ID NO: 525 - DNA, 27 bp, Homo sapiens
  source 1..27: mol_type = genomic DNA
aagctactattacctccaggcacggat

SEQ ID NO: 526 - DNA, 27 bp, Homo sapiens
  source 1..27: mol_type = genomic DNA
ccgtgccagccaaggacagggtggact

SEQ ID NO: 527 - DNA, 28 bp, Homo sapiens
  source 1..28: mol_type = genomic DNA
cacgcatccagcgccccttctccgtgaa

SEQ ID NO: 528 - DNA, 27 bp, Homo sapiens
  source 1..27: mol_type = genomic DNA
tgaaatccagacaattgaagatggggc

SEQ ID NO: 529 - DNA, 24 bp, Homo sapiens
  source 1..24: mol_type = genomic DNA
tctctgcaggcaagttgctccaga

SEQ ID NO: 530 - DNA, 23 bp, Homo sapiens
  source 1..23: mol_type = genomic DNA
tccaggctcccgcctgacaaaca

SEQ ID NO: 531 - DNA, 28 bp, Homo sapiens
  source 1..28: mol_type = genomic DNA
ctggtttccatccacatatgtggaagag

SEQ ID NO: 532 - DNA, 25 bp, Homo sapiens
  source 1..25: mol_type = genomic DNA
cggcgcgcttctcttatgggcgtct

SEQ ID NO: 533 - DNA, 27 bp, Homo sapiens
  source 1..27: mol_type = genomic DNA
aagacatggaagccagtgattatgagc

SEQ ID NO: 534 - DNA, 26 bp, Homo sapiens
  source 1..26: mol_type = genomic DNA
tggtggagaaaaatgcagatccagag

SEQ ID NO: 535 - DNA, 68 bp, Homo sapiens
  source 1..68: mol_type = genomic DNA
ggctgctttttaaatcttccgttcttcgaacctcactcatcacctctcggccagtgtcgggagccaga

SEQ ID NO: 536 - DNA, 65 bp, Homo sapiens
  source 1..65: mol_type = genomic DNA
ggatgttggaagctccttcatatatcgtaccaatctttgcatctcggaagtatttctccacaggg

SEQ ID NO: 537 - DNA, 62 bp, Homo sapiens
  source 1..62: mol_type = genomic DNA
tgtctttttgtcccattcccaccatcaccccctgatgtctgggacgtcccacaatggatggg

SEQ ID NO: 538 - DNA, 62 bp, Homo sapiens
  source 1..62: mol_type = genomic DNA
aatccttctgacccatgcccaccatcacgccctggtgcctggggcgccccacgatggagggg

SEQ ID NO: 539 - DNA, 75 bp, Homo sapiens
  source 1..75: mol_type = genomic DNA
attgtcaatgaccagcgcggcgatctcttcttccattgcgaccccgccttttgttcccggggaaggcgcgacgag

SEQ ID NO: 540 - DNA, 66 bp, Homo sapiens
  source 1..66: mol_type = genomic DNA
ggacacaaatcgcttctttcttatgcttccagttcctgtgggctgtcctacgccttgcagtgccgg

SEQ ID NO: 541 - DNA, 63 bp, Homo sapiens
  source 1..63: mol_type = genomic DNA
ccacagacattaacgtcaggatgtggttctgcaggtcggccccgtagaaggcagccatggacg

SEQ ID NO: 542 - DNA, 56 bp, Homo sapiens
  source 1..56: mol_type = genomic DNA
tggatgggccggggtccgacgacagcgcgagttggggcaggagcgcaaggcgggga

SEQ ID NO: 543 - DNA, 58 bp, Homo sapiens
  source 1..58: mol_type = genomic DNA
caacaactgtatggccagcattatttcctccctggcagcggcacacgatgtcggcgtc

SEQ ID NO: 544 - DNA, 64 bp, Homo sapiens
  source 1..64: mol_type = genomic DNA
cttgagagctttcttcatgttgtcaagcaacagagctgtatctgcaggttcgtaagcatagaga

SEQ ID NO: 545 - DNA, 77 bp, Homo sapiens
  source 1..77: mol_type = genomic DNA
actcgaagtttcttctcttccctcaaagttgcctgcaaaattgctttctccttaagtagagaaacttgctgcttaag

SEQ ID NO: 546 - DNA, 59 bp, Homo sapiens
  source 1..59: mol_type = genomic DNA
tcgtgggctccggggaggctgcctacgcagtgccttccgaaggtctgcgcgtccgtctg

SEQ ID NO: 547 - DNA, 77 bp, Homo sapiens
  source 1..77: mol_type = genomic DNA
accaaactgcaggaataactccaagtaatcatcaaaggtgcccaaataagttcccatttctttttccaggatgactt

SEQ ID NO: 548 - DNA, 66 bp, Homo sapiens
  source 1..66: mol_type = genomic DNA
tgaagcagctttgacagtacctcctttggttgccatggccatgactctaggtcaagatcagagttc

SEQ ID NO: 549 - DNA, 72 bp, Homo sapiens
  source 1..72: mol_type = genomic DNA
aaggcaacagcattgtttcaggatcgacatttttttctatcaccttgcggccgttcacgtagaagagcagct

SEQ ID NO: 550 - DNA, 58 bp, Homo sapiens
  source 1..58: mol_type = genomic DNA
gtggctggagaagggacctggagcttttctttcaagatgaaggcagtttccagatgca

SEQ ID NO: 551 - DNA, 56 bp, Homo sapiens
  source 1..56: mol_type = genomic DNA
tctcacaccaaggcagggtcctcttgtccaagggatcttcctctgacagagactga

SEQ ID NO: 552 - DNA, 61 bp, Homo sapiens
  source 1..61: mol_type = genomic DNA
acgataagggaggctgtgcctatgaactggtcaaagaagccattgatcatatccaagtgtc

SEQ ID NO: 553 - DNA, 76 bp, Homo sapiens
  source 1..76: mol_type = genomic DNA
ccgaggtccatagctgccaaccataaatgttgctttatccactttcaccccagtcctgtaggtgtgctgaacgtat

SEQ ID NO: 554 - DNA, 51 bp, Homo sapiens
  source 1..51: mol_type = genomic DNA
ttcctgttccctttgacaggggctgccatggcccggagaggtcccgcggcg

SEQ ID NO: 555 - DNA, 73 bp, Homo sapiens
  source 1..73: mol_type = genomic DNA
ttgagtggtgtccagttaacagaaataacaattttctctttaggctgcaacacgaaacagcgctgcgacacac

SEQ ID NO: 556 - DNA, 77 bp, Homo sapiens
  source 1..77: mol_type = genomic DNA
ttcttcctggcttcctcgaagtcttccttctggccaatgttggccagataggcaatgacgtcatagccttgttcctt

SEQ ID NO: 557 - DNA, 59 bp, Homo sapiens
  source 1..59: mol_type = genomic DNA
aacccagtcctttgggagcttttatggagactttgtaacacaggcatgattgattaatc

SEQ ID NO: 558 - DNA, 72 bp, Homo sapiens
  source 1..72: mol_type = genomic DNA
ccttgggctctagttcccgcctcgtcctcattttcctgttgtacatcttcagcaggatcagaaccacggtga

SEQ ID NO: 559 - DNA, 70 bp, Homo sapiens
  source 1..70: mol_type = genomic DNA
agaacagggccggcaccaggaggtacaagagccacatttctcaaggcccgtgttgaatcctgggctctcc

SEQ ID NO: 560 - DNA, 60 bp, Homo sapiens
  source 1..60: mol_type = genomic DNA
ttggcttgagggccaaggaaatattgactgattagatagaagagcacatgatagatctga

SEQ ID NO: 561 - DNA, 70 bp, Homo sapiens
  source 1..70: mol_type = genomic DNA
agccgcaagatgttgggggtgatgatagagtacatgggactccccagagccagggggaggtgggttagta

SEQ ID NO: 562 - DNA, 63 bp, Homo sapiens
  source 1..63: mol_type = genomic DNA
aacattaggtactggtggaaccagagctgttattttgtacatcatatcatttatgtgttgcaa

SEQ ID NO: 563 - DNA, 53 bp, Homo sapiens
  source 1..53: mol_type = genomic DNA
ttgactctggctcaaggtgggcttcctggaggcagcggcaaggaggcagttct

SEQ ID NO: 564 - DNA, 71 bp, Homo sapiens
  source 1..71: mol_type = genomic DNA
ttcttatccaagggcattataggaccattgtcttcctccctcatgaagacagacttgttcctgtcctcttt

SEQ ID NO: 565 - DNA, 54 bp, Homo sapiens
  source 1..54: mol_type = genomic DNA
atggtctctctccaagtcgctggtcatatcccttttctttccaggtgctccaac

SEQ ID NO: 566 - DNA, 57 bp, Homo sapiens
  source 1..57: mol_type = genomic DNA
acatttgatgaccaaatatgggtttacagtttcattggcatacttcttctccaggtc

SEQ ID NO: 567 - DNA, 63 bp, Homo sapiens
  source 1..63: mol_type = genomic DNA
ttcgttcctggtaatcatcaagcttaccctttttcttctccaggttccgaagtttcttgtcga

SEQ ID NO: 568 - DNA, 77 bp, Homo sapiens
  source 1..77: mol_type = genomic DNA
tgtgtcctgggaatggcaatggtgcctcatcaacataaatctgaaattcttcaattaagttacaaaaagttactcct

SEQ ID NO: 569 - DNA, 83 bp, Homo sapiens
  source 1..83: mol_type = genomic DNA
ctgatcttcaggagtttgctgcttgcatacttattcttgatggcgatgaatttagttaagttttcatttactttcaccacatt

SEQ ID NO: 570 - DNA, 62 bp, Homo sapiens
  source 1..62: mol_type = genomic DNA
aagatggaccggtcactggggcaggagaaactttgcccaaagacccctgtgtggggcagctg

SEQ ID NO: 571 - DNA, 57 bp, Homo sapiens
  source 1..57: mol_type = genomic DNA
ttatcccgccacgagcacagtttctttatctgtgtcctcgccagcacacacgccacc

SEQ ID NO: 572 - DNA, 60 bp, Homo sapiens
  source 1..60: mol_type = genomic DNA
ggtagcaggcattttctatgttgcaccctttgaagattctcccctcctgggtgagcaggg

SEQ ID NO: 573 - DNA, 60 bp, Homo sapiens
  source 1..60: mol_type = genomic DNA
tgatgaagtttctttacttaacctgacattgctactcaaaaacttgtacttttgggggaa

SEQ ID NO: 574 - DNA, 61 bp, Homo sapiens
  source 1..61: mol_type = genomic DNA
actctctgctcctgcattttgcacctctggacaaaggcctaaacttgagttatcaaaatag

SEQ ID NO: 575 - DNA, 75 bp, Homo sapiens
  source 1..75: mol_type = genomic DNA
ttgtactctggccagtggggcagcccttccccattggggtttccattgcgagcaaagttggcccagaatttcatc

SEQ ID NO: 576 - DNA, 74 bp, Homo sapiens
  source 1..74: mol_type = genomic DNA
tctctgccgcccaggatccgaccacggggcggcgccgcgcaggcggccgctcctaggaggaccagaactgccag

SEQ ID NO: 577 - DNA, 53 bp, Homo sapiens
  source 1..53: mol_type = genomic DNA
agcatattttccatctgccgtctctgcagctctcagtctggaagcagcaaagt

SEQ ID NO: 578 - DNA, 65 bp, Homo sapiens
  source 1..65: mol_type = genomic DNA
ccaataaacagagcggctcctaattcatacttttgctcaacaaagagaggatcaaagaattccgt

SEQ ID NO: 579 - DNA, 49 bp, Homo sapiens
  source 1..49: mol_type = genomic DNA
ttcattcacacgagcaagggcacctttctcagtctcgcagcccctgtgc

SEQ ID NO: 580 - DNA, 57 bp, Homo sapiens
  source 1..57: mol_type = genomic DNA
atgggtctcatagtcctctgggatggtgtcattgcagcggtaacgcaggttggccca

SEQ ID NO: 581 - DNA, 64 bp, Homo sapiens
  source 1..64: mol_type = genomic DNA
atctcctcctccagccgagacacggcatccgagctgggagtgccactggcctctggtgctgccc

SEQ ID NO: 582 - DNA, 74 bp, Homo sapiens
  source 1..74: mol_type = genomic DNA
agctccttccgatcactgatcacaaactccttagcgaaattctgtacgacctccttcaccagggtcttgtccgt

SEQ ID NO: 583 - DNA, 59 bp, Homo sapiens
  source 1..59: mol_type = genomic DNA
ataggtgaagttgccgaagtcatgctccctctgtgggtcggtgggagtttctcgcctcc

SEQ ID NO: 584 - DNA, 76 bp, Homo sapiens
  source 1..76: mol_type = genomic DNA
ttctctgaggctgatgaaggctggtctggaacaggcatagctcccaaaggcgcggcgcccggcggcttcctcgcaa

SEQ ID NO: 585 - DNA, 73 bp, Homo sapiens
  source 1..73: mol_type = genomic DNA
caatgcaattacctcggccacttcgtaagggtgcacagaacgaacaaaatctgtcaaagctgggaccaaggaa

SEQ ID NO: 586 - DNA, 59 bp, Homo sapiens
  source 1..59: mol_type = genomic DNA
tcccttctggtcagttggatttgtcactgttcagcatcttttcgatgattttcttaact

SEQ ID NO: 587 - DNA, 52 bp, Homo sapiens
  source 1..52: mol_type = genomic DNA
ttccgggagcacttgcatttggacccgtccacacgcgcggtgtacagcgcca

SEQ ID NO: 588 - DNA, 62 bp, Homo sapiens
  source 1..62: mol_type = genomic DNA
cgaagaatcaaagtcatatttcctttttcctatctggaatcgagctgcgtctgccgagaagc

SEQ ID NO: 589 - DNA, 56 bp, Homo sapiens
  source 1..56: mol_type = genomic DNA
ttgacagagacgacaaactgacagaccttcattcctgctgcggctgcagggccact

SEQ ID NO: 590 - DNA, 71 bp, Homo sapiens
  source 1..71: mol_type = genomic DNA
atcgtgaggcccagggaccggccgtcccccagcaccaggttcacctttttctcatcccctccttgcaggag

SEQ ID NO: 591 - DNA, 63 bp, Homo sapiens
  source 1..63: mol_type = genomic DNA
atttctcagtccggccccagagaacaatctttctggcgccgcgctccgcgaactcgcgggcga

SEQ ID NO: 592 - DNA, 71 bp, Homo sapiens
  source 1..71: mol_type = genomic DNA
tctccttgctattcctcatcacgaggctgggcctcctcctgttgttacagatgtgaaacaagcctctgtgc

SEQ ID NO: 593 - DNA, 79 bp, Homo sapiens
  source 1..79: mol_type = genomic DNA
aagaaggtggcattcagtagtgagacttttattatcaaatagttctgactgagaaattttagtttccccttcttctaag

SEQ ID NO: 594 - DNA, 75 bp, Homo sapiens
  source 1..75: mol_type = genomic DNA
tgtgctgtgctgctagctattccatggtcttcatcagtataccacattgcctggaaatccactccaacatcgacc

SEQ ID NO: 595 - DNA, 70 bp, Homo sapiens
  source 1..70: mol_type = genomic DNA
atcaaatcgctgcacctcccacgaaatggggttctgagctcccagaggggtccatgccccaaccagaagt

SEQ ID NO: 596 - DNA, 56 bp, Homo sapiens
  source 1..56: mol_type = genomic DNA
gcacccttctggaccaaagcgccaaggactgtgagggggacccaatctggactcct

SEQ ID NO: 597 - DNA, 55 bp, Homo sapiens
  source 1..55: mol_type = genomic DNA
aggtccaacaggaactggtagtgggcggggagccgcggcagcgccagtcccgcca

SEQ ID NO: 598 - DNA, 63 bp, Homo sapiens
  source 1..63: mol_type = genomic DNA
gaagaagtgtcaatagaagcaggtttgaagtcatagcgcacagtgtggaaggcgcagcgcggc

SEQ ID NO: 599 - DNA, 76 bp, Homo sapiens
  source 1..76: mol_type = genomic DNA
ttacacatctcagctccaaatggccagtcctctgccagcagcttgtagacattgatagggatgtcaatgacgatgt

SEQ ID NO: 600 - DNA, 56 bp, Homo sapiens
  source 1..56: mol_type = genomic DNA
atcccactcatatccgtcagtgcattgcgtgtacgtgatggtttcttcggtgtcct

SEQ ID NO: 601 - DNA, 69 bp, Homo sapiens
  source 1..69: mol_type = genomic DNA
caccttcaaaagcatgatgctcttcatggggtttataaaatactgctttaaaagttatgtggggcagaa

SEQ ID NO: 602 - DNA, 73 bp, Homo sapiens
  source 1..73: mol_type = genomic DNA
gtagtaacaacaagtgaattattagctgcctctaaaacacctgtgctgttactgctgcaaatactgggcagaa

SEQ ID NO: 603 - DNA, 63 bp, Homo sapiens
  source 1..63: mol_type = genomic DNA
gtgttctccaagaattgatctcaaatcaggttccctccagctccccggctaccgaagcgctag

SEQ ID NO: 604 - DNA, 71 bp, Homo sapiens
  source 1..71: mol_type = genomic DNA
acaccaggaatgacgaggtctgtttgaattctccttcacttcgggcactaggctggctgtaaatcaccttc

SEQ ID NO: 605 - DNA, 73 bp, Homo sapiens
  source 1..73: mol_type = genomic DNA
agatctctagagaaaacttcctcactgggtcggtcaagatcatcagaagtgtctgtctgtggagtgtatcctt

SEQ ID NO: 606 - DNA, 76 bp, Homo sapiens
  source 1..76: mol_type = genomic DNA
ccttcatccatcaacatttctgagtcaggtatacgtggggtcttatctggtgcatctacctcagggggttttgaag

SEQ ID NO: 607 - DNA, 57 bp, Homo sapiens
  source 1..57: mol_type = genomic DNA
attcccctttcctggagctgttactagttggttgttgctttaagtgtaataacccta

SEQ ID NO: 608 - DNA, 70 bp, Homo sapiens
  source 1..70: mol_type = genomic DNA
gataaaatcttctggtccattgttgctcatatcacagaactccgccacaaacttccaaaaagcccgctca

SEQ ID NO: 609 - DNA, 59 bp, Homo sapiens
  source 1..59: mol_type = genomic DNA
agctcctgcgcctcccggtcgtggttgtccttaactgctttgttgaatttggtacagaa

SEQ ID NO: 610 - DNA, 56 bp, Homo sapiens
  source 1..56: mol_type = genomic DNA
cttcgttaagcaacaacgcgcattgaaactcgagcgggctaaagcgctacggcgag

SEQ ID NO: 611 - DNA, 56 bp, Homo sapiens
  source 1..56: mol_type = genomic DNA
aacctgcgtcgctgtccttctcttccagcccgtcgtcgccctcgcccaccacatcg

SEQ ID NO: 612 - DNA, 62 bp, Homo sapiens
  source 1..62: mol_type = genomic DNA
ttcttcgcttgacggagccagcagttcccagcctgggcactgcggtcctccatgaactggca

SEQ ID NO: 613 - DNA, 56 bp, Homo sapiens
  source 1..56: mol_type = genomic DNA
tgctcccgcttctgccgcacttccagttctctctgaaagacctggacactgtcctt

SEQ ID NO: 614 - DNA, 58 bp, Homo sapiens
  source 1..58: mol_type = genomic DNA
tccatcgacaacccagtcatttccccaggtgaatgggctgcctccactcccctcttcc

SEQ ID NO: 615 - DNA, 75 bp, Homo sapiens
  source 1..75: mol_type = genomic DNA
agtcctgcgtttatccgaagctgccacgccctaagcaaacctcacttcttttccttagatgatgtgttttgcctg

SEQ ID NO: 616 - DNA, 70 bp, Homo sapiens
  source 1..70: mol_type = genomic DNA
tgacttaaggcaggatccttccattgagatgaatgtggattcgtcaccagcacgcagtgcaggtccgggg

SEQ ID NO: 617 - DNA, 53 bp, Homo sapiens
  source 1..53: mol_type = genomic DNA
tcttccaggcgtccgtgtgagggttcgtgaccaggagacaatgcaggtctcgg

SEQ ID NO: 618 - DNA, 75 bp, Homo sapiens
  source 1..75: mol_type = genomic DNA
tgaggtccaccaccctgttgctgtagccaaattcgttgtcataccaggaaatgagcttgacaaagtggtcgttga

SEQ ID NO: 619 - DNA, 61 bp, Homo sapiens
  source 1..61: mol_type = genomic DNA
aagtttgtccaagtcctgcccacttcttgcatgagtgtcttcataaatccatgcgcgccgc

SEQ ID NO: 620 - DNA, 62 bp, Homo sapiens
  source 1..62: mol_type = genomic DNA
aagcagggcagtcagcagctcctacctgccacgaggtgtgggggaccctggggtcccagctg

SEQ ID NO: 621 - DNA, 58 bp, Homo sapiens
  source 1..58: mol_type = genomic DNA
agccatgtccagggtgttgttccccagatcagagatcctttagcactggaaagaaggt

SEQ ID NO: 622 - DNA, 66 bp, Homo sapiens
  source 1..66: mol_type = genomic DNA
acagctttatttttatcaccagagttttaaataaatacacagttccatcagaccagcccccgagtc

SEQ ID NO: 623 - DNA, 58 bp, Homo sapiens
  source 1..58: mol_type = genomic DNA
tgaagggcaatgaaccaagtacaaagacacaccctcagtgcttcctatgaggaagccc

SEQ ID NO: 624 - DNA, 76 bp, Homo sapiens
  source 1..76: mol_type = genomic DNA
ttctccaggaagccccagtcacccatggctcccgggcctccgtcgcctgcctgccgggcggcccaggtggaggtgg

SEQ ID NO: 625 - DNA, 72 bp, Homo sapiens
  source 1..72: mol_type = genomic DNA
cgtcctacacacccgggtcgcagcattggaaacacttctctgggtgggcttatccaccatcttcttcagttt

SEQ ID NO: 626 - DNA, 68 bp, Homo sapiens
  source 1..68: mol_type = genomic DNA
gccacacagtaaaagatgaatatgaaaaatccttgtaaggtattaaagatggcaaacagatacatgaa

SEQ ID NO: 627 - DNA, 69 bp, Homo sapiens
  source 1..69: mol_type = genomic DNA
cccattgtacccgctgtatggtgacaccggcctcttagctgcaaccggctcatccatggaaaaggcctt

SEQ ID NO: 628 - DNA, 67 bp, Homo sapiens
  source 1..67: mol_type = genomic DNA
acgttttctgaagcataatgagtgagctcttcagctgttcaagcatcactatggagtctcggagcac

SEQ ID NO: 629 - DNA, 77 bp, Homo sapiens
  source 1..77: mol_type = genomic DNA
atgaggagttacttcatttcctccaataattttttcacagacatcttcaggaattagcaggagagaaacgacaactg

SEQ ID NO: 630 - DNA, 76 bp, Homo sapiens
  source 1..76: mol_type = genomic DNA
ttttcttgtcgttgctgctcactgtgcttttcaagatttcgttcagctccttcttcctcttctcctctttcacgtc

SEQ ID NO: 631 - DNA, 56 bp, Homo sapiens
  source 1..56: mol_type = genomic DNA
tggaacctagagccgaactcaagtttccattctcgtccgcactctccttctccacc

SEQ ID NO: 632 - DNA, 65 bp, Homo sapiens
  source 1..65: mol_type = genomic DNA
ggagaattcaatctaatcacagagctagtactttgccccgagtaattgttctcgctccccacgtc

SEQ ID NO: 633 - DNA, 59 bp, Homo sapiens
  source 1..59: mol_type = genomic DNA
tgtaggattctgcctctaggaaatgtgccatccttctgaataattggacccaggaagag

SEQ ID NO: 634 - DNA, 79 bp, Homo sapiens
  source 1..79: mol_type = genomic DNA
gttggtgaagtaacagtcagcctttgcctgaatcacaaaatcttctggagagtctgtgccttgagtcatggaggaatcc

SEQ ID NO: 635 - DNA, 68 bp, Homo sapiens
  source 1..68: mol_type = genomic DNA
ctcctgtttctccagatcattgttgctctcataatggaaggctttgaccttggcaatgagggtgccgg

SEQ ID NO: 636 - DNA, 74 bp, Homo sapiens
  source 1..74: mol_type = genomic DNA
aattgcttgcgcttttcccactgacccacgtttctcactgactctgtcttgaagcagccaggctggatgatgct

SEQ ID NO: 637 - DNA, 54 bp, Homo sapiens
  source 1..54: mol_type = genomic DNA
atgtcctggaggaactgagcagcatgtcctccaccagcagtctgctggatgccc

SEQ ID NO: 638 - DNA, 58 bp, Homo sapiens
  source 1..58: mol_type = genomic DNA
cctctccatccatggatgtctcacactgtctgctgtgataaaatccattcttgttgca

SEQ ID NO: 639 - DNA, 83 bp, Homo sapiens
  source 1..83: mol_type = genomic DNA
gatgttggctctcgagttgtagaagcatgtgaactgggaagtgccattcaccgctgcagatgcccaagaggtagccaggggca

SEQ ID NO: 640 - DNA, 62 bp, Homo sapiens
  source 1..62: mol_type = genomic DNA
aatgctaaccgccacagtcgggaatctgtgcacaaaattgcaggtgccgtcgatggggtcga

SEQ ID NO: 641 - DNA, 63 bp, Homo sapiens
  source 1..63: mol_type = genomic DNA
tgagccccaggcctcaggccccagccagccggccgccagcagcagaaggcaggcggcccccag

SEQ ID NO: 642 - DNA, 82 bp, Homo sapiens
  source 1..82: mol_type = genomic DNA
cgcggacgctaggcacaccagcttggagttagttcagcaaacccctttttcttgcagtgcgatttcaggtctggaacctcag

SEQ ID NO: 643 - DNA, 58 bp, Homo sapiens
  source 1..58: mol_type = genomic DNA
agtgcccagcagctcttccagagctccgggtggcaggcaggccctatgctctgcctgg

SEQ ID NO: 644 - DNA, 64 bp, Homo sapiens
  source 1..64: mol_type = genomic DNA
gccttctcctttttgaaacttttctatttcttggttcaccaggcgcagggcgtgcgtgaaggag

SEQ ID NO: 645 - DNA, 76 bp, Homo sapiens
  source 1..76: mol_type = genomic DNA
tattgaatgggcgctagctttccgctctgccaaattaaatggtctgcatctcaccaccacctggatgttcttcccc

SEQ ID NO: 646 - DNA, 73 bp, Homo sapiens
  source 1..73: mol_type = genomic DNA
gaatcaaatcttcttttgaagttacagccaagtttcctcagccgcgctgcagaccgacgggcggaccgggtca

SEQ ID NO: 647 - DNA, 67 bp, Homo sapiens
  source 1..67: mol_type = genomic DNA
atgttgttctgcagttcagccagagtctggtcctgtttgattaagatgtcatcacaagtggtcaagg

SEQ ID NO: 648 - DNA, 71 bp, Homo sapiens
  source 1..71: mol_type = genomic DNA
cacctcttccttcatgatcctatctcagcaccgtctcaaactaaatgtcccttccccgttctccctgggcc

SEQ ID NO: 649 - DNA, 76 bp, Homo sapiens
  source 1..76: mol_type = genomic DNA
atctgcacaggggaagtggaaccacaaaggaggagatgtgcgagtatcatagatgtagagatcattgcagatggtg

SEQ ID NO: 650 - DNA, 75 bp, Homo sapiens
  source 1..75: mol_type = genomic DNA
ctgcacagttaagttcagcattatctgagtcttttatctcatgtttgaaagccaaaccattcattgtcacccatg

SEQ ID NO: 651 - DNA, 57 bp, Homo sapiens
  source 1..57: mol_type = genomic DNA
agatctgggactgcagctctgtcaactccgtctcattgagggtcctgaggaagttga

SEQ ID NO: 652 - DNA, 74 bp, Homo sapiens
  source 1..74: mol_type = genomic DNA
actgcacagcgctgaccacagtggctgagggcgagtccatcctgccctcctcgccctccaccagcttcctgtag

SEQ ID NO: 653 - DNA, 57 bp, Homo sapiens
  source 1..57: mol_type = genomic DNA
cattcacagcttcaacaccttcacacagcctctgctcctcgccctccagcaggcgcc

SEQ ID NO: 654 - DNA, 77 bp, Homo sapiens
  source 1..77: mol_type = genomic DNA
atgatggcctggctgccccgcagcagctccaactccatgtctttcatcctgtccatcatctccatggtctccccaaa

SEQ ID NO: 655 - DNA, 77 bp, Homo sapiens
  source 1..77: mol_type = genomic DNA
cctcacacattcatgctgacaaacaagcacctgcatgtagtgatctgcaatagcttcatacagaccagccttatacc

SEQ ID NO: 656 - DNA, 58 bp, Homo sapiens
  source 1..58: mol_type = genomic DNA
agaaccaacagcaggggcacaactcctgccgccaagaccttcattatgggctgcactt

SEQ ID NO: 657 - DNA, 65 bp, Homo sapiens
  source 1..65: mol_type = genomic DNA
atctgtcttggtctccacttgcttgctttcatccatggacatctccctctgcataagtttcttgg

SEQ ID NO: 658 - DNA, 56 bp, Homo sapiens
  source 1..56: mol_type = genomic DNA
cttaccctggtctggaggccagaaccgaggaaagggctccctgcccctccaagtac

SEQ ID NO: 659 - DNA, 79 bp, Homo sapiens
  source 1..79: mol_type = genomic DNA
tttaactcccctgggtgtggagtggctcgccttagaagtgttctcgtctcattgtcttcttcatctttctcatcctcca

SEQ ID NO: 660 - DNA, 73 bp, Homo sapiens
  source 1..73: mol_type = genomic DNA
tgtagcactccacgccgttgggcgggtatgcactctcattacctgccgggtcgagcgcccgcgaggtgaggtt

SEQ ID NO: 661 - DNA, 59 bp, Homo sapiens
  source 1..59: mol_type = genomic DNA
aactacatttaaatcattaccaggaactgtttgttttgtagtgaaccttgagtatgtgc

SEQ ID NO: 662 - DNA, 75 bp, Homo sapiens
  source 1..75: mol_type = genomic DNA
ctctgatccccactgctgttctcttcaacattcaagttattaatcttgcgggtcctcttgccccgaattattgtc

SEQ ID NO: 663 - DNA, 64 bp, Homo sapiens
  source 1..64: mol_type = genomic DNA
actgcatcactgatctggtcacagatcttatccgggtgtccctctcccacagactccgatgtga

SEQ ID NO: 664 - DNA, 72 bp, Homo sapiens
  source 1..72: mol_type = genomic DNA
aattcacatgaggggttgatggtcctgatcgagaaaccacaacctgcatgaagcgaccctctgatgtcccaa

SEQ ID NO: 665 - DNA, 57 bp, Homo sapiens
  source 1..57: mol_type = genomic DNA
gtgagtagcccaacttcctttaaaacattcctgcgagcagaagtacgagccctggat

SEQ ID NO: 666 - DNA, 69 bp, Homo sapiens
  source 1..69: mol_type = genomic DNA
aagccttgctccatggactggctattttcatcaaatctccagtatttgtccgctgcaaagaagtatgtt

SEQ ID NO: 667 - DNA, 57 bp, Homo sapiens
  source 1..57: mol_type = genomic DNA
ggtcaggaaaaattgatggaaatagccctcaacaaagtcccatcctttatggtctgc

SEQ ID NO: 668 - DNA, 74 bp, Homo sapiens
  source 1..74: mol_type = genomic DNA
cgccagtagaagcggtcctggcagaaataggctttctctcggtactggaagacgtcgtgcgtgtccaaaggcac

SEQ ID NO: 669 - DNA, 62 bp, Homo sapiens
  source 1..62: mol_type = genomic DNA
attcctctcctgttccagctcctccaccttttgctggaacaaattcctttcagccaaaacac

SEQ ID NO: 670 - DNA, 74 bp, Homo sapiens
  source 1..74: mol_type = genomic DNA
agagtgcttgaggggctcattcaaaatcttgtcgttgaaatcggtgctgtcctccgactcgcggatcataaggg

SEQ ID NO: 671 - DNA, 58 bp, Homo sapiens
  source 1..58: mol_type = genomic DNA
gcagcagctgcacttctccgatgcccctttgcagatgcagccctgggcacacttggca

SEQ ID NO: 672 - DNA, 59 bp, Homo sapiens
  source 1..59: mol_type = genomic DNA
tccattgcaagccgaggtgagactggagttcccaagcgagaagagaagaggcagtggaa

SEQ ID NO: 673 - DNA, 56 bp, Homo sapiens
  source 1..56: mol_type = genomic DNA
tttgcagatgcagccctgggcacacttggcacagcccacagggcagcaggagcagc

SEQ ID NO: 674 - DNA, 62 bp, Homo sapiens
  source 1..62: mol_type = genomic DNA
tagagtcgggacaggttgcacgcgggttcgctgggacttggaggaggcgtggtggagtgcag

SEQ ID NO: 675 - DNA, 58 bp, Homo sapiens
  source 1..58: mol_type = genomic DNA
tgctgccaccattacctgcagaaaccttctcataggggctacgatcggtactgctagg

SEQ ID NO: 676 - DNA, 77 bp, Homo sapiens
  source 1..77: mol_type = genomic DNA
caacattgtaggcttctttggtattggtttttttttaaaggaataacaatcccttgatgtggcaagaatagattgta

SEQ ID NO: 677 - DNA, 66 bp, Homo sapiens
  source 1..66: mol_type = genomic DNA
atcatgccctccaggtattcgtctgtggggttcttccccagcgaggccagcatgtcgtgcaggtcc

SEQ ID NO: 678 - DNA, 70 bp, Homo sapiens
  source 1..70: mol_type = genomic DNA
tcaattgccgactcattgctgatctggacatgcagataaatgttgtcaaaagtaccatctttttcacaga

SEQ ID NO: 679 - DNA, 63 bp, Homo sapiens
  source 1..63: mol_type = genomic DNA
gttcctcctgtagaggtgaattaagtaatacttcctgggccttctttcgaagcagccacttgt

SEQ ID NO: 680 - DNA, 63 bp, Homo sapiens
  source 1..63: mol_type = genomic DNA
ttgcacccttgcaggaaggcgtcgggccagctgctcgatgtgcatattctccaggagcgcgct

SEQ ID NO: 681 - DNA, 56 bp, Homo sapiens
  source 1..56: mol_type = genomic DNA
actgaactgcgcttcatgcttatgaccttttttccagtttcctgacacgacccagg

SEQ ID NO: 682 - DNA, 76 bp, Homo sapiens
  source 1..76: mol_type = genomic DNA
tgcatgtcctcgaactgaaacagtggctggaagcaagatttatagttgagtcccacatcgtggtaggtaaggatcg

SEQ ID NO: 683 - DNA, 74 bp, Homo sapiens
  source 1..74: mol_type = genomic DNA
tggatggaatttttcaaaaatttcaccatatgttttcttatcttcttcaggaaaatcctctggatgtaatttca

SEQ ID NO: 684 - DNA, 54 bp, Homo sapiens
  source 1..54: mol_type = genomic DNA
acagtgagcacccaggctcagggcacctgtacagagcaagaggatagctgagac

SEQ ID NO: 685 - DNA, 63 bp, Homo sapiens
  source 1..63: mol_type = genomic DNA
caagcttttcgtagtcctcaggagtcatcttggcatcgtgcacgaccttgcgggtgtgcttgg

SEQ ID NO: 686 - DNA, 61 bp, Homo sapiens
  source 1..61: mol_type = genomic DNA
tcttcatcttcttcaacttgggccgggtggcgcagtcagtgcacaggatcttgcccacctc

SEQ ID NO: 687 - DNA, 69 bp, Homo sapiens
  source 1..69: mol_type = genomic DNA
tgccagctctcctcagggttggtgggcagcacttgagtgagttcagtgcccatcaggatgaggaagagg

SEQ ID NO: 688 - DNA, 79 bp, Homo sapiens
  source 1..79: mol_type = genomic DNA
ggttttgatctttccagcgaaaaccgacgaaattcagctccaaacttgctcttcacctccatagtgcccaggcagccgc

SEQ ID NO: 689 - DNA, 59 bp, Homo sapiens
  source 1..59: mol_type = genomic DNA
ccttccattgtgaaagccactctcagtccagagtctcaccgcctggaaggaaaggtcgg

SEQ ID NO: 690 - DNA, 71 bp, Homo sapiens
  source 1..71: mol_type = genomic DNA
ggcagtttaccttcacattccattacgcaagccaggaagttgatgtcggccgggcgcactaggcggtagct

SEQ ID NO: 691 - DNA, 83 bp, Homo sapiens
  source 1..83: mol_type = genomic DNA
catctcctcaaactgggtttgacttcgtagcccttccaaaggaattgtattaagaagtaacaatactttcatacagaggaact

SEQ ID NO: 692 - DNA, 59 bp, Homo sapiens
  source 1..59: mol_type = genomic DNA
actggttcaggtaagcagaccatcttttctctgtcattgacaggcaaaagggcagtgca

SEQ ID NO: 693 - DNA, 61 bp, Homo sapiens
  source 1..61: mol_type = genomic DNA
aaaaaggaaaaacacacagcactgaagggtctctgggtggtaatgccagcgtgggctgggg

SEQ ID NO: 694 - DNA, 62 bp, Homo sapiens
  source 1..62: mol_type = genomic DNA
agaccggccagtgggcgcgagaaagacagctgctgagagagacagacggggccaggccagcg

SEQ ID NO: 695 - DNA, 77 bp, Homo sapiens
  source 1..77: mol_type = genomic DNA
agatctgggcaaagaggctggtcttcaccaaccagagcagcacactcgatgtcactccatacagactcagagtcctg

SEQ ID NO: 696 - DNA, 54 bp, Homo sapiens
  source 1..54: mol_type = genomic DNA
ctggctgtggggcgcatttttactctctggttcccgctggaagatgacgacccg

SEQ ID NO: 697 - DNA, 59 bp, Homo sapiens
  source 1..59: mol_type = genomic DNA
cacacaaggtacacctgtagttcttctgacctgtatgtatcttgaggtgggtccgcagg

SEQ ID NO: 698 - DNA, 73 bp, Homo sapiens
  source 1..73: mol_type = genomic DNA
ttttggattcatatgccttctgtaagaattttctcaaagtatcttctgggaaatcacgcggctgtaccacata

SEQ ID NO: 699 - DNA, 63 bp, Homo sapiens
  source 1..63: mol_type = genomic DNA
atttggcccgtgtagcttccctttgagggtgtgtgacttgccatctgcaaaagtcatggccaa

SEQ ID NO: 700 - DNA, 63 bp, Homo sapiens
  source 1..63: mol_type = genomic DNA
atggctgggctttcgcctgggggaagccactgtcgcgtctcgcagtcctcagactgggagtca

SEQ ID NO: 701 - DNA, 63 bp, Homo sapiens
  source 1..63: mol_type = genomic DNA
aaactgtgcaggattgcagtccagacatcttgtcatcccaggccgccagccgggctctctgag

SEQ ID NO: 702 - DNA, 70 bp, Homo sapiens
  source 1..70: mol_type = genomic DNA
tacaattcctccaactctgctgccatctccttctctcctacgagctcctggaaggaggtgtagggtttca

SEQ ID NO: 703 - DNA, 63 bp, Homo sapiens
  source 1..63: mol_type = genomic DNA
tctgacctatccctggtagtaagaactcttggaacccccttttcaaatgctactgccacattt

SEQ ID NO: 704 - DNA, 79 bp, Homo sapiens
  source 1..79: mol_type = genomic DNA
gccctcttcaatcttttcaagctctttgaatttataaccaatgcctcttccaatgtctttgccttccaaattctttaat

SEQ ID NO: 705 - DNA, 66 bp, Homo sapiens
  source 1..66: mol_type = genomic DNA
gcaaaattggacagctgtctcatagttcttcaccgtccccccttctgaccctggtgtgcctgtggt

SEQ ID NO: 706 - DNA, 58 bp, Homo sapiens
  source 1..58: mol_type = genomic DNA
gtacataacacttccaattcagccaaactctggaagtgcagcgccatcttcccaggag

SEQ ID NO: 707 - DNA, 59 bp, Homo sapiens
  source 1..59: mol_type = genomic DNA
cctgcacaagaagaattctctccataaatctgggaaggcgtatgttcaaggtacggatt

SEQ ID NO: 708 - DNA, 68 bp, Homo sapiens
  source 1..68: mol_type = genomic DNA
atttccccaaacgtccctcaccttcctgaagtaaagactctgggttgtagcgctctgtgctgaagacc

SEQ ID NO: 709 - DNA, 55 bp, Homo sapiens
  source 1..55: mol_type = genomic DNA
gaaggaaaagaagaggtcaaatggacaggagagagcggagattggttgttctcag

SEQ ID NO: 710 - DNA, 60 bp, Homo sapiens
  source 1..60: mol_type = genomic DNA
cccatcattgtcgattcgatcaacaatcttccctagcctctccttgctctcgtccggggt

SEQ ID NO: 711 - DNA, 63 bp, Homo sapiens
  source 1..63: mol_type = genomic DNA
gcacacaactgcttcaaatggtaggatgctcttcatgaaggtcacgatgtacatgaggcgggg

SEQ ID NO: 712 - DNA, 59 bp, Homo sapiens
  source 1..59: mol_type = genomic DNA
aatataatctccttcccgggctcctgccaccgaggcagagcagtaaggatccaggaagt

SEQ ID NO: 713 - DNA, 78 bp, Homo sapiens
  source 1..78: mol_type = genomic DNA
aatgaatgggtcctctgcagagccatcagtatcttagaggtgcccaggaggaagaatcttacaaaaatctggcagttt

SEQ ID NO: 714 - DNA, 62 bp, Homo sapiens
  source 1..62: mol_type = genomic DNA
aatgacacctgcacaattctccgagtgctttcaagcaacttcgggaggcagtgactaagacc

SEQ ID NO: 715 - DNA, 65 bp, Homo sapiens
  source 1..65: mol_type = genomic DNA
agcctagagttgatcgactccagcgactttttcgtcttctttgcggccaccatcttcctgcctta

SEQ ID NO: 716 - DNA, 71 bp, Homo sapiens
  source 1..71: mol_type = genomic DNA
taggagtcctcaatagtggggtcgtagtcagacacgaagtaggactggatgaactggatggtcagcgcgct

SEQ ID NO: 717 - DNA, 70 bp, Homo sapiens
  source 1..70: mol_type = genomic DNA
tccttcatcaccttgtccacagcatccacatccttctgggcatccaggaagccagagagctccgtctgca

SEQ ID NO: 718 - DNA, 75 bp, Homo sapiens
  source 1..75: mol_type = genomic DNA
acatcatttcttgtcatcaatagcagggattttccatcaatttcctgttcctgaaaagcactagcttgctcctca

SEQ ID NO: 719 - DNA, 58 bp, Homo sapiens
  source 1..58: mol_type = genomic DNA
aggagctcacgagacactccttcttcttctcccgagtcttcttcaggatgaagatgat

SEQ ID NO: 720 - DNA, 59 bp, Homo sapiens
  source 1..59: mol_type = genomic DNA
actgcatgaccagggctggcaagaagctgtgtaacagagggctgcctttagtttgtggc

SEQ ID NO: 721 - DNA, 58 bp, Homo sapiens
  source 1..58: mol_type = genomic DNA
tccaccacagctttgtgcaccatctcagacacctggatatttgagtggttgctgatgc

SEQ ID NO: 722 - DNA, 68 bp, Homo sapiens
  source 1..68: mol_type = genomic DNA
gtagcatttggatttgaggaggctctatccccagccagcagcagcagcaggagggtcagcagggtcag

SEQ ID NO: 723 - DNA, 57 bp, Homo sapiens
  source 1..57: mol_type = genomic DNA
accaaacagatgactctgcgacagcgttcgctctgcatgtaccgggccaccccttcc

SEQ ID NO: 724 - DNA, 75 bp, Homo sapiens
  source 1..75: mol_type = genomic DNA
acaatgaaggcaatgctcagtggatagttggagccacagattgtcggagatggcttctttggagggctaggtggt

SEQ ID NO: 725 - DNA, 67 bp, Homo sapiens
  source 1..67: mol_type = genomic DNA
aagtaatagttcaaatagcagccgttaatattaccaaagtctgtgtgactgctcatccatccgatgg

SEQ ID NO: 726 - DNA, 73 bp, Homo sapiens
  source 1..73: mol_type = genomic DNA
aaagcatcaccaaggacgttgaccatggtcctgaaccggtccaggagccagtcgacagcaatgatcagggtga

SEQ ID NO: 727 - DNA, 70 bp, Homo sapiens
  source 1..70: mol_type = genomic DNA
atgaggcccagggaacactgtagtcatcctgtgttcacctccgtcccgaaacggttgtgtctgcatctgc

SEQ ID NO: 728 - DNA, 69 bp, Homo sapiens
  source 1..69: mol_type = genomic DNA
tccaggccaagatctctttgtatactaaccggcaaaggagcaagcaggctaggacgtcggcagagatga

SEQ ID NO: 729 - DNA, 58 bp, Homo sapiens
  source 1..58: mol_type = genomic DNA
gtagataccaaaatggaagcttgacacccctgttagctcagcaagcagagacgatcac

SEQ ID NO: 730 - DNA, 77 bp, Homo sapiens
  source 1..77: mol_type = genomic DNA
accagcttctttcattgctttcctactgttttccacaaactccatcagcactttatccatatagaattctctgccag

SEQ ID NO: 731 - DNA, 79 bp, Homo sapiens
  source 1..79: mol_type = genomic DNA
attttcttgtgtccacttttctgtctggaggatcccagtcatgcttttctgttgaagaccgatctcttggtcgaagcgg

SEQ ID NO: 732 - DNA, 55 bp, Homo sapiens
  source 1..55: mol_type = genomic DNA
tggttcagggataggatagttctccaggcgcaagtcccccggtccgtgcaccacc

SEQ ID NO: 733 - DNA, 52 bp, Homo sapiens
  source 1..52: mol_type = genomic DNA
actcgagaccctcgggccaagggtaggctcccagcagcgaagccatggccgc

SEQ ID NO: 734 - DNA, 51 bp, Homo sapiens
  source 1..51: mol_type = genomic DNA
ttcaccttcttaccgactcccaaggcaaactcatcaatctcgtggtctcgt

SEQ ID NO: 735 - DNA, 55 bp, Homo sapiens
  source 1..55: mol_type = genomic DNA
agtctattggcttccgggggctgcgggacctccgctcgccagggggtggcttctt

SEQ ID NO: 736 - DNA, 65 bp, Homo sapiens
  source 1..65: mol_type = genomic DNA
tagaacaagtgaggacagcacgcagtgaatctactccagccacgttgcccggcggtgttggtgag

SEQ ID NO: 737 - DNA, 64 bp, Homo sapiens
  source 1..64: mol_type = genomic DNA
atcctggtcagctcctcgttctctttagtcttctgctccactgtcttctccagcgactggatgc

SEQ ID NO: 738 - DNA, 73 bp, Homo sapiens
  source 1..73: mol_type = genomic DNA
ttggagccatcagggtacaggctgttcaccagcttgctcagaatcacgccattcttcagccagacctggaagc

SEQ ID NO: 739 - DNA, 70 bp, Homo sapiens
  source 1..70: mol_type = genomic DNA
aaggggttcatgtcattgaaggcgatgttcatcagcttccggctgttggagatggtcttggtgaagaagc

SEQ ID NO: 740 - DNA, 61 bp, Homo sapiens
  source 1..61: mol_type = genomic DNA
aagctctcccgagcttacatctgacaatctgcttttcacattgtatttgatttgttggatc

SEQ ID NO: 741 - DNA, 66 bp, Homo sapiens
  source 1..66: mol_type = genomic DNA
gtcctcatatatgaagttgttatggttacagaaagaaaataaatatttgtgcacacagagatagca

SEQ ID NO: 742 - DNA, 59 bp, Homo sapiens
  source 1..59: mol_type = genomic DNA
cggaaatgcagcaaatcttgtttaaatatctctgcattcgtacttgaggtctgagaaat

SEQ ID NO: 743 - DNA, 63 bp, Homo sapiens
  source 1..63: mol_type = genomic DNA
ttcttccccaccaccttggcccggatcacgatgtcggagttgcagaaggcgtcctgggggtgg

SEQ ID NO: 744 - DNA, 57 bp, Homo sapiens
  source 1..57: mol_type = genomic DNA
acacttgttttgccaggttttaggatcacagtgtggtaagcgcagctccacaggctt

SEQ ID NO: 745 - DNA, 72 bp, Homo sapiens
  source 1..72: mol_type = genomic DNA
cccttggattaccttcttgaactgatcttctagatcgcaagtcaagactgccatcatgttcccccaaatgca

SEQ ID NO: 746 - DNA, 61 bp, Homo sapiens
  source 1..61: mol_type = genomic DNA
ccagtataggatgcaagaactacatacacaaaggtcatcaatggtgagattattgacagca

SEQ ID NO: 747 - DNA, 71 bp, Homo sapiens
  source 1..71: mol_type = genomic DNA
aagtccatatggaagtcatcactctcccccttggatttcttgcttgtgactgctttcgaaacaattttctc

SEQ ID NO: 748 - DNA, 62 bp, Homo sapiens
  source 1..62: mol_type = genomic DNA
agacaaagaccgagatccacacggagacgacggagaaacacagggcagacacacacgaaagg

SEQ ID NO: 749 - DNA, 75 bp, Homo sapiens
  source 1..75: mol_type = genomic DNA
aagtccgccatcccacatctgtttaatttctccccatatgaagcccaggacccacggtaatatcatccactcgac

SEQ ID NO: 750 - DNA, 68 bp, Homo sapiens
  source 1..68: mol_type = genomic DNA
gggtgatgtacagcagcgtcagcagcacccccaggaactggggaagcaggatgcccaggaggatgccc

SEQ ID NO: 751 - DNA, 76 bp, Homo sapiens
  source 1..76: mol_type = genomic DNA
aaagtgtgtccttgactccatggagtaattcttgtagttttgcttggcagattccaaaagtttgatggcctcttcg

SEQ ID NO: 752 - DNA, 55 bp, Homo sapiens
  source 1..55: mol_type = genomic DNA
attgtagcttgccaatggaacatatcatctccaacaggacctgctgaacactgtg

SEQ ID NO: 753 - DNA, 53 bp, Homo sapiens
  source 1..53: mol_type = genomic DNA
tatcctccatccagacctagtgggagaggcagagcctgaagtgccagcagcga

SEQ ID NO: 754 - DNA, 79 bp, Homo sapiens
  source 1..79: mol_type = genomic DNA
aagatatctagattctggggtggtctcgattttaaaagcttgagaagctgcaaacattatccaaagtatatttgaggct

SEQ ID NO: 755 - DNA, 58 bp, Homo sapiens
  source 1..58: mol_type = genomic DNA
tggtgtaggtcttgattctgctaaccggcagtcgctgggtagtgaggctcacacaggt

SEQ ID NO: 756 - DNA, 60 bp, Homo sapiens
  source 1..60: mol_type = genomic DNA
tgtaaagtgaaatgagctggctggctggagacggacagggtgccagagactactagccag

SEQ ID NO: 757 - DNA, 55 bp, Homo sapiens
  source 1..55: mol_type = genomic DNA
aaaaatcctcagattaccaacagatctcctgagcggcggtgagatccgcggctgc

SEQ ID NO: 758 - DNA, 56 bp, Homo sapiens
  source 1..56: mol_type = genomic DNA
tacgtcttcatcccactgtgcagcttcctgtgctgctccacagcctcgttatcagg

SEQ ID NO: 759 - DNA, 65 bp, Homo sapiens
  source 1..65: mol_type = genomic DNA
tctacaacagcaccttttgaaatataaaactttacaagatccagtctgttgttaatagcagccca

SEQ ID NO: 760 - DNA, 69 bp, Homo sapiens
  source 1..69: mol_type = genomic DNA
tgagtatttaagtgcttcttcattacaaaagcaaccccacagacatgacacttgtattccctcatccca